European Patent Application EP 4 647 489 A1, published November 12, 2025. Title: Bacteria Secreting Interleukin-10. Applicant: Synthetica Pioneering Co., Ltd. The sequence listing filed with the application follows.

SEQUENCE LISTING (98 sequences)

SEQ ID NO: 1 - DNA, 5922 bp, synthetic construct
  source 1..5922: mol_type = other DNA
tggcgaatgggacgcgccctgtagcggcgcattaagcgcggcgggtgtggtggttacgcgcagcgtgaccgctacacttgccagcgccctagcgcccgctcctttcgctttcttcccttcctttctcgccacgttcgccggctttccccgtcaagctctaaatcgggggctccctttagggttccgatttagtgctttacggcacctcgaccccaaaaaacttgattagggtgatggttcacgtagtgggccatcgccctgatagacggtttttcgccctttgacgttggagtccacgttctttaatagtggactcttgttccaaactggaacaacactcaaccctatctcggtctattcttttgatttataagggattttgccgatttcggcctattggttaaaaaatgagctgatttaacaaaaatttaacgcgaattttaacaaaatattaacgtttacaatttcaggtggcacttttcggggaaatgtgcgcggaacccctatttgtttatttttctaaatacattcaaatatgtatccgctcatgagacaataaccctgataaatgcttcaataatattgaaaaaggaagagtatgagtattcaacatttccgtgtcgcccttattcccttttttgcggcattttgccttcctgtttttgctcacccagaaacgctggtgaaagtaaaagatgctgaagatcagttgggtgcacgagtgggttacatcgaactggatctcaacagcggtaagatccttgagagttttcgccccgaagaacgttttccaatgatgagcacttttaaagttctgctatgtggcgcggtattatcccgtattgacgccgggcaagagcaactcggtcgccgcatacactattctcagaatgacttggttgagtactcaccagtcacagaaaagcatcttacggatggcatgacagtaagagaattatgcagtgctgccataaccatgagtgataacactgcggccaacttacttctgacaacgatcggaggaccgaaggagctaaccgcttttttgcacaacatgggggatcatgtaactcgccttgatcgttgggaaccggagctgaatgaagccataccaaacgacgagcgtgacaccacgatgcctgcagcaatggcaacaacgttgcgcaaactattaactggcgaactacttactctagcttcccggcaacaattaatagactggatggaggcggataaagttgcaggaccacttctgcgctcggcccttccggctggctggtttattgctgataaatctggagccggtgagcgtgggtctcgcggtatcattgcagcactggggccagatggtaagccctcccgtatcgtagttatctacacgacggggagtcaggcaactatggatgaacgaaatagacagatcgctgagataggtgcctcactgattaagcattggtaactgtcagaccaagtttactcatatatactttagattgatttaaaacttcatttttaatttaaaaggatctaggtgaagatcctttttgataatctcatgaccaaaatcccttaacgtgagttttcgttccactgagcgtcagaccccgtagaaaagatcaaaggatcttcttgagatcctttttttctgcgcgtaatctgctgcttgcaaacaaaaaaaccaccgctaccagcggtggtttgtttgccggatcaagagctaccaactctttttccgaaggtaactggcttcagcagagcgcagataccaaatactgtccttctagtgtagccgtagttaggccaccacttcaagaactctgtagcaccgcctacatacctcgctctgctaatcctgttaccagtggctgctgccagtggcgataagtcgtgtcttaccgggttggactcaagacgatagttaccggataaggcgcagcggtcgggctgaacggggggttcgtgcacacagcccagcttggagcgaacgacctacaccgaactgagatacctacagcgtgagctatgagaaagcgccacgcttcccgaagggagaaaggcggacaggtatccggtaagcggcagggtcggaacaggagagcgcacgagggagcttccagggggaaacgcctggtatctttatagtcctgtcgggtttcgccacctctgacttgagcgtcgatttttgtgatgctcgtcaggggggcggagcctatggaaaaacgccagcaacgcggcctttttacggttcctggccttttgctggccttttgctcacatgttctttcctgcgttatcccctgattctgtggataaccgtattaccgcctttgagtgagctgataccgctcgccgcagccgaacgaccgagcgcagcgagtcagtgagcgaggaagcggaagagcgcctgatgcggtattttctccttacgcatctgtgcggtatttcacaccgcatatatggtgcactctcagtacaatctgctctgatgccgcatagttaagccagtatacactccgctatcgctacgtgactgggtcatggctgcgccccgacacccgccaacacccgctgacgcgccctgacgggcttgtctgctcccggcatccgcttacagacaagctgtgaccgtctccgggagctgcatgtgtcagaggttttcaccgtcatcaccgaaacgcgcgaggcagctgcggtaaagctcatcagcgtggtcgtgaagcgattcacagatgtctgcctgttcatccgcgtccagctcgttgagtttctccagaagcgttaatgtctggcttctgataaagcgggccatgttaagggcggttttttcctgtttggtcactgatgcctccgtgtaagggggatttctgttcatgggggtaatgataccgatgaaacgagagaggatgctcacgatacgggttactgatgatgaacatgcccggttactggaacgttgtgagggtaaacaactggcggtatggatgcggcgggaccagagaaaaatcactcagggtcaatgccagcgcttcgttaatacagatgtaggtgttccacagggtagccagcagcatcctgcgatgcagatccggaacataatggtgcagggcgctgacttccgcgtttccagactttacgaaacacggaaaccgaagaccattcatgttgttgctcaggtcgcagacgttttgcagcagcagtcgcttcacgttcgctcgcgtatcggtgattcattctgctaaccagtaaggcaaccccgccagcctagccgggtcctcaacgacaggagcacgatcatgcgcacccgtggggccgccatgccggcgataatggcctgcttctcgccgaaacgtttggtggcgggaccagtgacgaaggcttgagcgagggcgtgcaagattccgaataccgcaagcgacaggccgatcatcgtcgcgctccagcgaaagcggtcctcgccgaaaatgacccagagcgctgccggcacctgtcctacgagttgcatgataaagaagacagtcataagtgcggcgacgatagtcatgccccgcgcccaccggaaggagctgactgggttgaaggctctcaagggcatcggtcgagatcccggtgcctaatgagtgagctaacttacattaattgcgttgcgctcactgcccgctttccagtcgggaaacctgtcgtgccagctgcattaatgaatcggccaacgcgcggggagaggcggtttgcgtattgggcgccagggtggtttttcttttcaccagtgagacgggcaacagctgattgcccttcaccgcctggccctgagagagttgcagcaagcggtccacgctggtttgccccagcaggcgaaaatcctgtttgatggtggttaacggcgggatataacatgagctgtcttcggtatcgtcgtatcccactaccgagatatccgcaccaacgcgcagcccggactcggtaatggcgcgcattgcgcccagcgccatctgatcgttggcaaccagcatcgcagtgggaacgatgccctcattcagcatttgcatggtttgttgaaaaccggacatggcactccagtcgccttcccgttccgctatcggctgaatttgattgcgagtgagatatttatgccagccagccagacgcagacgcgccgagacagaacttaatgggcccgctaacagcgcgatttgctggtgacccaatgcgaccagatgctccacgcccagtcgcgtaccgtcttcatgggagaaaataatactgttgatgggtgtctggtcagagacatcaagaaataacgccggaacattagtgcaggcagcttccacagcaatggcatcctggtcatccagcggatagttaatgatcagcccactgacgcgttgcgcgagaagattgtgcaccgccgctttacaggcttcgacgccgcttcgttctaccatcgacaccaccacgctggcacccagttgatcggcgcgagatttaatcgccgcgacaatttgcgacggcgcgtgcagggccagactggaggtggcaacgccaatcagcaacgactgtttgcccgccagttgttgtgccacgcggttgggaatgtaattcagctccgccatcgccgcttccactttttcccgcgttttcgcagaaacgtggctggcctggttcaccacgcgggaaacggtctgataagagacaccggcatactctgcgacatcgtataacgttactggtttcacattcaccaccctgaattgactctcttccgggcgctatcatgccataccgcgaaaggttttgcgccattcgatggtgtccgggatctcgacgctctcccttatgcgactcctgcattaggaagcagcccagtagtaggttgaggccgttgagcaccgccgccgcaaggaatggtgcatgcaaggagatggcgcccaacagtcccccggccacggggcctgccaccatacccacgccgaaacaagcgctcatgagcccgaagtggcgagcccgatcttccccatcggtgatgtcggcgatataggcgccagcaaccgcacctgtggcgccggtgatgccggccacgatgcgtccggcgtagaggatcgagatctcgatcccgcgaaattaatacgactcactataggggaattgtgagcggataacaattcccctctagaaataattttgtttaactttaagaaggagatatacatatgaaatacctgctgccgaccgctgctgctggtctgctgctcctcgctgcccagccggcgatggccgatgatgatgatgatagccgcggccagtacagccgcgaggacaataactgcacccattttccggtgggccagagccatatgctgctggaactgcgcaccgcgtttagccaagttaagacgttcttccagaccaaagaccagctggataacattttactgaccgactctttaatgcaagattttaagggctatctgggctgccaagctttaagcgagatgatccagttctatttagtggaagtgatgccgcaagctgaaaaacacggcccggagatcaaagaacatttaaactctttaggcgagaaactgaagactttacgcatgcgtttacgtcgttgccatcgctttctgccgtgcgagaacaaaagcaaagcggtggagcaagttaagagcgacttcaacaaactgcaagatcaaggtgtgtataaggcgatgaacgaattcgatatctttatcaactgcatcgaagcgtatatgatgattaaaatgaaaagccaccaccaccaccaccactgagatccggctgctaacaaagcccgaaaggaagctgagttggctgctgccaccgctgagcaataactagcataaccccttggggcctctaaacgggtcttgaggggttttttgctgaaaggaggaactatatccggat

SEQ ID NO: 2 - DNA, 4978 bp, synthetic construct
  source 1..4978: mol_type = other DNA
ctaaattgtaagcgttaatattttgttaaaattcgcgttaaatttttgttaaatcagctcattttttaaccaataggccgaaatcggcaaaatcccttataaatcaaaagaatagaccgagatagggttgagtgttgttccagtttggaacaagagtccactattaaagaacgtggactccaacgtcaaagggcgaaaaaccgtctatcagggcgatggcccactacgtgaaccatcaccctaatcaagttttttggggtcgaggtgccgtaaagcactaaatcggaaccctaaagggagcccccgatttagagcttgacggggaaagccggcgaacgtggcgagaaaggaagggaagaaagcgaaaggagcgggcgctagggcgctggcaagtgtagcggtcacgctgcgcgtaaccaccacacccgccgcgcttaatgcgccgctacagggcgcgtcccattcgccattcaggctgcgcaactgttgggaagggcgatcggtgcgggcctcttcgctattacgccagctggcgaaagggggatgtgctgcaaggcgattaagttgggtaacgccagggttttcccagtcacgacgttgtaaaacgacggccagtgagcgcgcgtaatacgactcactataggcctctagaaataattttgtttaactttaagaaggagatatacaatgaaaaaacgctggttttggtttgtgctggcgctgattgtgctgtttccgtttcagagcagctttgcgaaccagagcccgggtcagggtacgcagagcgaaaacagctgtacgcattttccgggtaacctgccgaatatgctgcgtgatctgcgtgatgcatttagccgtgtgaaaacattttttcagatgaaagatcagctggataatctgctgctgaaagaaagcctgctggaagattttaaaggttatctgggttgtcaggccctgagcgaaatgattcagttttatctggaagaagttatgccgcaggcagaaaatcaggatcctgatattaaagcacatgttaatagcctgggtgaaaatctgaaaacactgcgtctgcgtctgcgccgttgccatcgctttctgccgtgtgaaaatggcggtggcagcggcggcaaaagcaaagcagtggaacaggttaaaaacgcatttaataaactgcaggaaaaaggtatctataaagccatgtcagaatttgatatctttatcaattatatcgaagcatatatgaccatgaaaatccgtaatcaccaccaccatcaccactaactcgagcaccaccaccaccaccactgagatccggctgctaacaaagcccgaaaggaagctgagttggctgctgccaccgctgagcaataactagcataaccccttggggcctctaaacgggtcttgaggggttttttgctgaaaggaggaactatatccggattggcgaatggggcgaattgggtaccgggccccccctcgagccgatcatattcaataacccttaatataacttcgtataatgtatgctatacgaagttattaggtctgaagaggagtttacgtcccatatggagtcccgcccaatgcttaatcagtgaggcacctatctcagcgatctgtctatttcgttcatccatagttgcctgactccccgtcgtgtagataactacgatacgggagggcttaccatctggccccagtgctgcaatgataccgcgagacccacgctcaccggctccagatttatcagcaataaaccagccagccggaagggccgagcgcagaagtggtcctgcaactttatccgcctccatccagtctattaattgttgccgggaagctagagtaagtagttcgccagttaatagtttgcgcaacgttgttgccattgctacaggcatcgtggtgtcacgctcgtcgtttggtatggcttcattcagctccggttcccaacgatcaaggcgagttacatgatcccccatgttgtgcaaaaaagcggttagctccttcggtcctccgatcgttgtcagaagtaagttggccgcagtgttatcactcatggttatggcagcactgcataattctcttactgtcatgccatccgtaagatgcttttctgtgactggtgagtactcaaccaagtcattctgagaatagtgtatgcggcgaccgagttgctcttgcccggcgtcaatacgggataataccgcgccacatagcagaactttaaaagtgctcatcattggaaaacgttcttcggggcgaaaactctcaaggatcttaccgctgttgagatccagttcgatgtaacccactcgtgcacccaactgatcttcagcatcttttactttcaccagcgtttctgggtgagcaaaaacaggaaggcaaaatgccgcaaaaaagggaataagggcgacacggaaatgttgaatactcatgcgaaacgatcctcatcctgtctcttgatcagatcctgatcccctgcgccatcagatccttggcggcaagaaagccatccagtttactttgcagggcttcccaaccttaccagagggcgccccagctggcaattccgacgtcattgcgttgctagccaagcttaggatccggaacccttaatataacttcgtataatgtatgctatacgaagttattaggtccctcgaagaggttcactagtcctcgaggtcgacggtatcgataagcttgatatcgaattcctgcagcccgggggatccactagttctagagcggccgccaccgcggtggagctccagcttttgttccctttagtgagggttaattgcgcgcttggcgtaatcatggtcatagctgtttcctgtgtgaaattgttatccgctcacaattccacacaacatacgagccggaagcataaagtgtaaagcctggggtgcctaatgagtgagctaactcacattaattgcgttgcgctcactgcccgctttccagtcgggaaacctgtcgtgccagctgcattaatgaatcggccaacgcgcggggagaggcggtttgcgtattgggcgctcttccgcttcctcgctcactgactcgctgcgctcggtcgttcggctgcggcgagcggtatcagctcactcaaaggcggtaatacggttatccacagaatcaggggataacgcaggaaagaacatgtgagcaaaaggccagcaaaaggccaggaaccgtaaaaaggccgcgttgctggcgtttttccataggctccgcccccctgacgagcatcacaaaaatcgacgctcaagtcagaggtggcgaaacccgacaggactataaagataccaggcgtttccccctggaagctccctcgtgcgctctcctgttccgaccctgccgcttaccggatacctgtccgcctttctcccttcgggaagcgtggcgctttctcatagctcacgctgtaggtatctcagttcggtgtaggtcgttcgctccaagctgggctgtgtgcacgaaccccccgttcagcccgaccgctgcgccttatccggtaactatcgtcttgagtccaacccggtaagacacgacttatcgccactggcagcagccactggtaacaggattagcagagcgaggtatgtaggcggtgctacagagttcttgaagtggtggcctaactacggctacactagaaggacagtatttggtatctgcgctctgctgaagccagttaccttcggaaaaagagttggtagctcttgatccggcaaacaaaccaccgctggtagcggtggtttttttgtttgcaagcagcagattacgcgcagaaaaaaaggatctcaagaagatcctttgatcttttctacggggtctgacgctcagtggaacgaaaactcacgttaagggattttggtcatgagattatcaaaaaggatcttcacctagatccttttaaattaaaaatgaagttttaaatcaatctaaagtatatatgagtaaacttggtctgacagttaccaatgcttaatcagtgaggcacctatctcagcgatctgtctatttcgttcatccatagttgcctgactccccgtcgtgtagataactacgatacgggagggcttaccatctggccccagtgctgcaatgataccgcgagacccacgctcaccggctccagatttatcagcaataaaccagccagccggaagggccgagcgcagaagtggtcctgcaactttatccgcctccatccagtctattaattgttgccgggaagctagagtaagtagttcgccagttaatagtttgcgcaacgttgttgccattgctacaggcatcgtggtgtcacgctcgtcgtttggtatggcttcattcagctccggttcccaacgatcaaggcgagttacatgatcccccatgttgtgcaaaaaagcggttagctccttcggtcctccgatcgttgtcagaagtaagttggccgcagtgttatcactcatggttatggcagcactgcataattctcttactgtcatgccatccgtaagatgcttttctgtgactggtgagtactcaaccaagtcattctgagaatagtgtatgcggcgaccgagttgctcttgcccggcgtcaatacgggataataccgcgccacatagcagaactttaaaagtgctcatcattggaaaacgttcttcggggcgaaaactctcaaggatcttaccgctgttgagatccagttcgatgtaacccactcgtgcacccaactgatcttcagcatcttttactttcaccagcgtttctgggtgagcaaaaacaggaaggcaaaatgccgcaaaaaagggaataagggcgacacggaaatgttgaatactcatactcttcctttttcaatattattgaagcatttatcagggttattgtctcatgagcggatacatatttgaatgtatttagaaaaataaacaaataggggttccgcgcacatttccccgaaaagtgccac

SEQ ID NO: 3 - DNA, 5922 bp, synthetic construct
  source 1..5922: mol_type = other DNA
tggcgaatgggacgcgccctgtagcggcgcattaagcgcggcgggtgtggtggttacgcgcagcgtgaccgctacacttgccagcgccctagcgcccgctcctttcgctttcttcccttcctttctcgccacgttcgccggctttccccgtcaagctctaaatcgggggctccctttagggttccgatttagtgctttacggcacctcgaccccaaaaaacttgattagggtgatggttcacgtagtgggccatcgccctgatagacggtttttcgccctttgacgttggagtccacgttctttaatagtggactcttgttccaaactggaacaacactcaaccctatctcggtctattcttttgatttataagggattttgccgatttcggcctattggttaaaaaatgagctgatttaacaaaaatttaacgcgaattttaacaaaatattaacgtttacaatttcaggtggcacttttcggggaaatgtgcgcggaacccctatttgtttatttttctaaatacattcaaatatgtatccgctcatgagacaataaccctgataaatgcttcaataatattgaaaaaggaagagtatgagtattcaacatttccgtgtcgcccttattcccttttttgcggcattttgccttcctgtttttgctcacccagaaacgctggtgaaagtaaaagatgctgaagatcagttgggtgcacgagtgggttacatcgaactggatctcaacagcggtaagatccttgagagttttcgccccgaagaacgttttccaatgatgagcacttttaaagttctgctatgtggcgcggtattatcccgtattgacgccgggcaagagcaactcggtcgccgcatacactattctcagaatgacttggttgagtactcaccagtcacagaaaagcatcttacggatggcatgacagtaagagaattatgcagtgctgccataaccatgagtgataacactgcggccaacttacttctgacaacgatcggaggaccgaaggagctaaccgcttttttgcacaacatgggggatcatgtaactcgccttgatcgttgggaaccggagctgaatgaagccataccaaacgacgagcgtgacaccacgatgcctgcagcaatggcaacaacgttgcgcaaactattaactggcgaactacttactctagcttcccggcaacaattaatagactggatggaggcggataaagttgcaggaccacttctgcgctcggcccttccggctggctggtttattgctgataaatctggagccggtgagcgtgggtctcgcggtatcattgcagcactggggccagatggtaagccctcccgtatcgtagttatctacacgacggggagtcaggcaactatggatgaacgaaatagacagatcgctgagataggtgcctcactgattaagcattggtaactgtcagaccaagtttactcatatatactttagattgatttaaaacttcatttttaatttaaaaggatctaggtgaagatcctttttgataatctcatgaccaaaatcccttaacgtgagttttcgttccactgagcgtcagaccccgtagaaaagatcaaaggatcttcttgagatcctttttttctgcgcgtaatctgctgcttgcaaacaaaaaaaccaccgctaccagcggtggtttgtttgccggatcaagagctaccaactctttttccgaaggtaactggcttcagcagagcgcagataccaaatactgtccttctagtgtagccgtagttaggccaccacttcaagaactctgtagcaccgcctacatacctcgctctgctaatcctgttaccagtggctgctgccagtggcgataagtcgtgtcttaccgggttggactcaagacgatagttaccggataaggcgcagcggtcgggctgaacggggggttcgtgcacacagcccagcttggagcgaacgacctacaccgaactgagatacctacagcgtgagctatgagaaagcgccacgcttcccgaagggagaaaggcggacaggtatccggtaagcggcagggtcggaacaggagagcgcacgagggagcttccagggggaaacgcctggtatctttatagtcctgtcgggtttcgccacctctgacttgagcgtcgatttttgtgatgctcgtcaggggggcggagcctatggaaaaacgccagcaacgcggcctttttacggttcctggccttttgctggccttttgctcacatgttctttcctgcgttatcccctgattctgtggataaccgtattaccgcctttgagtgagctgataccgctcgccgcagccgaacgaccgagcgcagcgagtcagtgagcgaggaagcggaagagcgcctgatgcggtattttctccttacgcatctgtgcggtatttcacaccgcatatatggtgcactctcagtacaatctgctctgatgccgcatagttaagccagtatacactccgctatcgctacgtgactgggtcatggctgcgccccgacacccgccaacacccgctgacgcgccctgacgggcttgtctgctcccggcatccgcttacagacaagctgtgaccgtctccgggagctgcatgtgtcagaggttttcaccgtcatcaccgaaacgcgcgaggcagctgcggtaaagctcatcagcgtggtcgtgaagcgattcacagatgtctgcctgttcatccgcgtccagctcgttgagtttctccagaagcgttaatgtctggcttctgataaagcgggccatgttaagggcggttttttcctgtttggtcactgatgcctccgtgtaagggggatttctgttcatgggggtaatgataccgatgaaacgagagaggatgctcacgatacgggttactgatgatgaacatgcccggttactggaacgttgtgagggtaaacaactggcggtatggatgcggcgggaccagagaaaaatcactcagggtcaatgccagcgcttcgttaatacagatgtaggtgttccacagggtagccagcagcatcctgcgatgcagatccggaacataatggtgcagggcgctgacttccgcgtttccagactttacgaaacacggaaaccgaagaccattcatgttgttgctcaggtcgcagacgttttgcagcagcagtcgcttcacgttcgctcgcgtatcggtgattcattctgctaaccagtaaggcaaccccgccagcctagccgggtcctcaacgacaggagcacgatcatgcgcacccgtggggccgccatgccggcgataatggcctgcttctcgccgaaacgtttggtggcgggaccagtgacgaaggcttgagcgagggcgtgcaagattccgaataccgcaagcgacaggccgatcatcgtcgcgctccagcgaaagcggtcctcgccgaaaatgacccagagcgctgccggcacctgtcctacgagttgcatgataaagaagacagtcataagtgcggcgacgatagtcatgccccgcgcccaccggaaggagctgactgggttgaaggctctcaagggcatcggtcgagatcccggtgcctaatgagtgagctaacttacattaattgcgttgcgctcactgcccgctttccagtcgggaaacctgtcgtgccagctgcattaatgaatcggccaacgcgcggggagaggcggtttgcgtattgggcgccagggtggtttttcttttcaccagtgagacgggcaacagctgattgcccttcaccgcctggccctgagagagttgcagcaagcggtccacgctggtttgccccagcaggcgaaaatcctgtttgatggtggttaacggcgggatataacatgagctgtcttcggtatcgtcgtatcccactaccgagatatccgcaccaacgcgcagcccggactcggtaatggcgcgcattgcgcccagcgccatctgatcgttggcaaccagcatcgcagtgggaacgatgccctcattcagcatttgcatggtttgttgaaaaccggacatggcactccagtcgccttcccgttccgctatcggctgaatttgattgcgagtgagatatttatgccagccagccagacgcagacgcgccgagacagaacttaatgggcccgctaacagcgcgatttgctggtgacccaatgcgaccagatgctccacgcccagtcgcgtaccgtcttcatgggagaaaataatactgttgatgggtgtctggtcagagacatcaagaaataacgccggaacattagtgcaggcagcttccacagcaatggcatcctggtcatccagcggatagttaatgatcagcccactgacgcgttgcgcgagaagattgtgcaccgccgctttacaggcttcgacgccgcttcgttctaccatcgacaccaccacgctggcacccagttgatcggcgcgagatttaatcgccgcgacaatttgcgacggcgcgtgcagggccagactggaggtggcaacgccaatcagcaacgactgtttgcccgccagttgttgtgccacgcggttgggaatgtaattcagctccgccatcgccgcttccactttttcccgcgttttcgcagaaacgtggctggcctggttcaccacgcgggaaacggtctgataagagacaccggcatactctgcgacatcgtataacgttactggtttcacattcaccaccctgaattgactctcttccgggcgctatcatgccataccgcgaaaggttttgcgccattcgatggtgtccgggatctcgacgctctcccttatgcgactcctgcattaggaagcagcccagtagtaggttgaggccgttgagcaccgccgccgcaaggaatggtgcatgcaaggagatggcgcccaacagtcccccggccacggggcctgccaccatacccacgccgaaacaagcgctcatgagcccgaagtggcgagcccgatcttccccatcggtgatgtcggcgatataggcgccagcaaccgcacctgtggcgccggtgatgccggccacgatgcgtccggcgtagaggatcgagatctcgatcccgcgaaattaatacgactcactataggggaattgtgagcggataacaattcccctctagaaataattttgtttaactttaagaaggagatatacatatgaaatacctgctgccgaccgctgctgctggtctgctgctcctcgctgcccagccggcgatggccgatgatgatgatgatagcccgggtcagggtacgcagagcgaaaacagctgtacgcattttccgggtaacctgccgaatatgctgcgtgatctgcgtgatgcatttagccgtgtgaaaacattttttcagatgaaagatcagctggataatctgctgctgaaagaaagcctgctggaagattttaaaggttatctgggttgtcaggccctgagcgaaatgattcagttttatctggaagaagttatgccgcaggcagaaaatcaggatcctgatattaaagcacatgttaatagcctgggtgaaaatctgaaaacactgcgtctgcgtctgcgccgttgccatcgctttctgccgtgtgaaaataaaagcaaagcagtggaacaggttaaaaacgcatttaataaactgcaggaaaaaggtatctataaagccatgtcagaatttgatatctttatcaattatatcgaagcatatatgaccatgaaaatccgtaatcaccaccaccaccaccactgagatccggctgctaacaaagcccgaaaggaagctgagttggctgctgccaccgctgagcaataactagcataaccccttggggcctctaaacgggtcttgaggggttttttgctgaaaggaggaactatatccggat

SEQ ID NO: 4 - DNA, 5907 bp, synthetic construct
  source 1..5907: mol_type = other DNA
tggcgaatgggacgcgccctgtagcggcgcattaagcgcggcgggtgtggtggttacgcgcagcgtgaccgctacacttgccagcgccctagcgcccgctcctttcgctttcttcccttcctttctcgccacgttcgccggctttccccgtcaagctctaaatcgggggctccctttagggttccgatttagtgctttacggcacctcgaccccaaaaaacttgattagggtgatggttcacgtagtgggccatcgccctgatagacggtttttcgccctttgacgttggagtccacgttctttaatagtggactcttgttccaaactggaacaacactcaaccctatctcggtctattcttttgatttataagggattttgccgatttcggcctattggttaaaaaatgagctgatttaacaaaaatttaacgcgaattttaacaaaatattaacgtttacaatttcaggtggcacttttcggggaaatgtgcgcggaacccctatttgtttatttttctaaatacattcaaatatgtatccgctcatgagacaataaccctgataaatgcttcaataatattgaaaaaggaagagtatgagtattcaacatttccgtgtcgcccttattcccttttttgcggcattttgccttcctgtttttgctcacccagaaacgctggtgaaagtaaaagatgctgaagatcagttgggtgcacgagtgggttacatcgaactggatctcaacagcggtaagatccttgagagttttcgccccgaagaacgttttccaatgatgagcacttttaaagttctgctatgtggcgcggtattatcccgtattgacgccgggcaagagcaactcggtcgccgcatacactattctcagaatgacttggttgagtactcaccagtcacagaaaagcatcttacggatggcatgacagtaagagaattatgcagtgctgccataaccatgagtgataacactgcggccaacttacttctgacaacgatcggaggaccgaaggagctaaccgcttttttgcacaacatgggggatcatgtaactcgccttgatcgttgggaaccggagctgaatgaagccataccaaacgacgagcgtgacaccacgatgcctgcagcaatggcaacaacgttgcgcaaactattaactggcgaactacttactctagcttcccggcaacaattaatagactggatggaggcggataaagttgcaggaccacttctgcgctcggcccttccggctggctggtttattgctgataaatctggagccggtgagcgtgggtctcgcggtatcattgcagcactggggccagatggtaagccctcccgtatcgtagttatctacacgacggggagtcaggcaactatggatgaacgaaatagacagatcgctgagataggtgcctcactgattaagcattggtaactgtcagaccaagtttactcatatatactttagattgatttaaaacttcatttttaatttaaaaggatctaggtgaagatcctttttgataatctcatgaccaaaatcccttaacgtgagttttcgttccactgagcgtcagaccccgtagaaaagatcaaaggatcttcttgagatcctttttttctgcgcgtaatctgctgcttgcaaacaaaaaaaccaccgctaccagcggtggtttgtttgccggatcaagagctaccaactctttttccgaaggtaactggcttcagcagagcgcagataccaaatactgtccttctagtgtagccgtagttaggccaccacttcaagaactctgtagcaccgcctacatacctcgctctgctaatcctgttaccagtggctgctgccagtggcgataagtcgtgtcttaccgggttggactcaagacgatagttaccggataaggcgcagcggtcgggctgaacggggggttcgtgcacacagcccagcttggagcgaacgacctacaccgaactgagatacctacagcgtgagctatgagaaagcgccacgcttcccgaagggagaaaggcggacaggtatccggtaagcggcagggtcggaacaggagagcgcacgagggagcttccagggggaaacgcctggtatctttatagtcctgtcgggtttcgccacctctgacttgagcgtcgatttttgtgatgctcgtcaggggggcggagcctatggaaaaacgccagcaacgcggcctttttacggttcctggccttttgctggccttttgctcacatgttctttcctgcgttatcccctgattctgtggataaccgtattaccgcctttgagtgagctgataccgctcgccgcagccgaacgaccgagcgcagcgagtcagtgagcgaggaagcggaagagcgcctgatgcggtattttctccttacgcatctgtgcggtatttcacaccgcatatatggtgcactctcagtacaatctgctctgatgccgcatagttaagccagtatacactccgctatcgctacgtgactgggtcatggctgcgccccgacacccgccaacacccgctgacgcgccctgacgggcttgtctgctcccggcatccgcttacagacaagctgtgaccgtctccgggagctgcatgtgtcagaggttttcaccgtcatcaccgaaacgcgcgaggcagctgcggtaaagctcatcagcgtggtcgtgaagcgattcacagatgtctgcctgttcatccgcgtccagctcgttgagtttctccagaagcgttaatgtctggcttctgataaagcgggccatgttaagggcggttttttcctgtttggtcactgatgcctccgtgtaagggggatttctgttcatgggggtaatgataccgatgaaacgagagaggatgctcacgatacgggttactgatgatgaacatgcccggttactggaacgttgtgagggtaaacaactggcggtatggatgcggcgggaccagagaaaaatcactcagggtcaatgccagcgcttcgttaatacagatgtaggtgttccacagggtagccagcagcatcctgcgatgcagatccggaacataatggtgcagggcgctgacttccgcgtttccagactttacgaaacacggaaaccgaagaccattcatgttgttgctcaggtcgcagacgttttgcagcagcagtcgcttcacgttcgctcgcgtatcggtgattcattctgctaaccagtaaggcaaccccgccagcctagccgggtcctcaacgacaggagcacgatcatgcgcacccgtggggccgccatgccggcgataatggcctgcttctcgccgaaacgtttggtggcgggaccagtgacgaaggcttgagcgagggcgtgcaagattccgaataccgcaagcgacaggccgatcatcgtcgcgctccagcgaaagcggtcctcgccgaaaatgacccagagcgctgccggcacctgtcctacgagttgcatgataaagaagacagtcataagtgcggcgacgatagtcatgccccgcgcccaccggaaggagctgactgggttgaaggctctcaagggcatcggtcgagatcccggtgcctaatgagtgagctaacttacattaattgcgttgcgctcactgcccgctttccagtcgggaaacctgtcgtgccagctgcattaatgaatcggccaacgcgcggggagaggcggtttgcgtattgggcgccagggtggtttttcttttcaccagtgagacgggcaacagctgattgcccttcaccgcctggccctgagagagttgcagcaagcggtccacgctggtttgccccagcaggcgaaaatcctgtttgatggtggttaacggcgggatataacatgagctgtcttcggtatcgtcgtatcccactaccgagatatccgcaccaacgcgcagcccggactcggtaatggcgcgcattgcgcccagcgccatctgatcgttggcaaccagcatcgcagtgggaacgatgccctcattcagcatttgcatggtttgttgaaaaccggacatggcactccagtcgccttcccgttccgctatcggctgaatttgattgcgagtgagatatttatgccagccagccagacgcagacgcgccgagacagaacttaatgggcccgctaacagcgcgatttgctggtgacccaatgcgaccagatgctccacgcccagtcgcgtaccgtcttcatgggagaaaataatactgttgatgggtgtctggtcagagacatcaagaaataacgccggaacattagtgcaggcagcttccacagcaatggcatcctggtcatccagcggatagttaatgatcagcccactgacgcgttgcgcgagaagattgtgcaccgccgctttacaggcttcgacgccgcttcgttctaccatcgacaccaccacgctggcacccagttgatcggcgcgagatttaatcgccgcgacaatttgcgacggcgcgtgcagggccagactggaggtggcaacgccaatcagcaacgactgtttgcccgccagttgttgtgccacgcggttgggaatgtaattcagctccgccatcgccgcttccactttttcccgcgttttcgcagaaacgtggctggcctggttcaccacgcgggaaacggtctgataagagacaccggcatactctgcgacatcgtataacgttactggtttcacattcaccaccctgaattgactctcttccgggcgctatcatgccataccgcgaaaggttttgcgccattcgatggtgtccgggatctcgacgctctcccttatgcgactcctgcattaggaagcagcccagtagtaggttgaggccgttgagcaccgccgccgcaaggaatggtgcatgcaaggagatggcgcccaacagtcccccggccacggggcctgccaccatacccacgccgaaacaagcgctcatgagcccgaagtggcgagcccgatcttccccatcggtgatgtcggcgatataggcgccagcaaccgcacctgtggcgccggtgatgccggccacgatgcgtccggcgtagaggatcgagatctcgatcccgcgaaattaatacgactcactataggggaattgtgagcggataacaattcccctctagaaataattttgtttaactttaagaaggagatatacatatgaaatacctgctgccgaccgctgctgctggtctgctgctcctcgctgcccagccggcgatggccagcccgggtcagggtacgcagagcgaaaacagctgtacgcattttccgggtaacctgccgaatatgctgcgtgatctgcgtgatgcatttagccgtgtgaaaacattttttcagatgaaagatcagctggataatctgctgctgaaagaaagcctgctggaagattttaaaggttatctgggttgtcaggccctgagcgaaatgattcagttttatctggaagaagttatgccgcaggcagaaaatcaggatcctgatattaaagcacatgttaatagcctgggtgaaaatctgaaaacactgcgtctgcgtctgcgccgttgccatcgctttctgccgtgtgaaaataaaagcaaagcagtggaacaggttaaaaacgcatttaataaactgcaggaaaaaggtatctataaagccatgtcagaatttgatatctttatcaattatatcgaagcatatatgaccatgaaaatccgtaatcaccaccaccaccaccactgagatccggctgctaacaaagcccgaaaggaagctgagttggctgctgccaccgctgagcaataactagcataaccccttggggcctctaaacgggtcttgaggggttttttgctgaaaggaggaactatatccggat

SEQ ID NO: 5 - DNA, 582 bp, synthetic construct
  source 1..582: mol_type = other DNA
atgaaatacctgctgccgaccgctgctgctggtctgctgctcctcgctgcccagccggcgatggccgatgatgatgatgatagcccgggtcagggtacgcagagcgaaaacagctgtacgcattttccgggtaacctgccgaatatgctgcgtgatctgcgtgatgcatttagccgtgtgaaaacattttttcagatgaaagatcagctggataatctgctgctgaaagaaagcctgctggaagattttaaaggttatctgggttgtcaggccctgagcgaaatgattcagttttatctggaagaagttatgccgcaggcagaaaatcaggatcctgatattaaagcacatgttaatagcctgggtgaaaatctgaaaacactgcgtctgcgtctgcgccgttgccatcgctttctgccgtgtgaaaataaaagcaaagcagtggaacaggttaaaaacgcatttaataaactgcaggaaaaaggtatctataaagccatgtcagaatttgatatctttatcaattatatcgaagcatatatgaccatgaaaatccgtaatcaccaccaccaccaccactga

SEQ ID NO: 6 - DNA, 4927 bp, synthetic construct
  source 1..4927: mol_type = other DNA
gtcttgaggggttttttgctgaaaggaggaactatatccggattggcgaatggggcgaattgggtaccgggccccccctcgagccgatcatattcaataacccttaatataacttcgtataatgtatgctatacgaagttattaggtctgaagaggagtttacgtcccatatggagtcccgcttaatcagcttgcttacgcaggaatgctgggatatccagataatccggctctttcgcagtttgcggcgcattgtcattcacgactttagcaaccggcttctgctcctgggtcagcggagccatcccgtgctgctggtagcgatccatcactggctgctgaacctgcttattagtcaccagagtgatttcaggacgtttgtccatgccgatacctgtcgcaacaacagttacgcgcagctcgtcattcatatccgggtcaagagaagtaccgataaccacggtcgcgttgtcggaagcaaatgcacggatggtgttacctaccgtttcgaactcatccagacgcaggtcgaagcccgctgtgatgtttaccagtacgccgcgtgcgccagacaggtcgatatcttccagcagcggagaagagatagccatttcagcagcttcttccgcacgatcttcaccgctcgccacaccagaacccatcattgcgtagcccatttcagacattacggtgcgtacgtctgcaaagtccacgttcatcaaacccggacgagtaatcagttcggcgataccttgcacagcgccttttagtacatcgttcgctgcgccaaacgcatccagcagggagataccacggcccagaactttcagcagtttgtcgttcgggatagtgatcagagagtccacatgcttggacagttcagtgatcccctgctccgcgaatgccatacgcttcttgccttcaaagttgaaaggcttagtgacgacagcaacggtcaggatacccaaatcttttgccacttcagcgacgactggtgctgcacctgtaccggtaccaccacccatacccgcagcaataaagaccatgtctgcaccttccagcgccgcacgcagtgcatcgcgatcctcatcagccgcattgcggccaacttctggattagcgccagcgcccagtcctttggtgataccgctaccgatttgaatcgtctgtccaaccgctgttttacgcagcgcttgtgcatcggtatttaccgcgaagaattcaacaccttcaatgcgctcacgcaccatgtgttcaacagcattaccgccgccgccgccgacgccgatgactttaatcaccgcgtcattggtaagttccattggttcaaacatagatcatcgacccctcattttattgccagatcagaagaactcgtcaagaaggcgatagaaggcgatgcgctgcgaatcgggagcggcgataccgtaaagcacgaggaagcggtcagcccattcgccgccaagctcttcagcaatatcacgggtagccaacgctatgtcctgatagcggtccgccacacccagccggccacagtcgatgaatccagaaaagcggccattttccaccatgatattcggcaagcaggcatcgccatgggtcacgacgagatcctcgccgtcgggcatgcgcgccttgagcctggcgaacagttcggccggcgcgagcccctgatgctcttcgtccagatcatcctgatcgacaagaccggcttccatccgagtacgtgctcgctcgatgcgatgtttcgcttggtggtcgaatgggcaggtagccggatcaagcgtatgcagccgccgcattgcatcagccatgatggatactttctcggcaggagcaaggtgagatgacaggagatcctgccccggcacttcgcccaatagcagccagtcccttcccgcttcagtgacaacgtcgagcacagctgcgcaaggaacgcccgtcgtggccagccacgatagccgcgctgcctcgtcctgcagttcattcagggcaccggacaggtcggtcttgacaaaaagaaccgggcgcccctgcgctgacagccggaacacggcggcatcagagcagccgattgtctgttgtgcccagtcatagccgaatagcctctccacccaagcggccggagaacctgcgtgcaatccatcttgttcaatcatgcgaaacgatcctcatcctgtctcttgatcagatcctgatcccctgcgccatcagatccttggcggcaagaaagccatccagtttactttgcagggcttcccaaccttaccagagggcgccccagctggcaattccactagaggacttcgattaggccaaataggccgttcagatccttccgtatttagccagtatgttctctagtgtggttcgttgtttttgcgtgagccatgagaacgaaccattgagatcatgcttactttgcatgtcactcaaaaattttgcctcaaaactggtgagctgaatttttgcagttaaagcatcgtgtagtgtttttcttagtccgttacgtaggtaggaatctgatgtaatggttgttggtattttgtcaccattcatttttatctggttgttctcaagttcggttacgagatccatttgtctatctagttcaacttggaaaatcaacgtatcagtcgggcggcctcgcttatcaaccaccaatttcatattgctgtaagtgtttaaatctttacttattggtttcaaaacccattggttaagccttttaaactcatggtagttattttcaagcattaacatgaacttaaattcatcaaggctaatctctatatttgccttgtgagttttcttttgtgttagttcttttaataaccactcataaatcctcatagagtatttgttttcaaaagacttaacatgttccagattatattttatgaatttttttaactggaaaagataaggcaatatctcttcactaaaaactaattctaatttttcgcttgagaacttggcatagtttgtccactggaaaatctcaaagcctttaaccaaaggattcctgatttccacagttctcgtcatcagctctctggttgctttagctaatacaccataagcattttccctactgatgttcatcatctgagcgtattggttataagtgaacgataccgtccgttctttccttgtagggttttcaatcgtggggttgagtagtgccacacagcataaaattagcttggtttcatgctccgttaagtcatagcgactaatcgctagttcatttgctttgaaaacaactaattcagacatacatctcaattggtctaggtgattttaatcactataccaattgagatgggctagtcaatgataattactagtccttttcctttgagttgtgggtatctgtaaattctgctagacctttgctggaaaacttgtaaattctgctagaccctctgtaaattccgctagacctttgtgtgttttttttgtttatattcaagtggttataatttatagaataaagaaagaataaaaaaagataaaaagaatagatcccagccctgtgtataactcactactttagtcagttccgcagtattacaaaaggatgtcgcaaacgctgtttgctcctctacaaaacagaccttaaaaccctaaaggcttaagtagcaccctcgcaagctcgggcaaatcgctgaatattccttttgtctccgaccatcaggcacctgagtcgctgtctttttcgtgacattcagttcgctgcgctcacggctctggcagtgaatgggggtaaatggcactacaggcgccttttatggattcatgcaaggaaactacccataatacaagaaaagcccgtcacgggcttctcagggcgttttatggcgggtctgctatgtggtgctatctgactttttgctgttcagcagttcctgccctctgattttccagtctgaccacttcggattatcccgtgacaggtcattcagactggctaatgcacccagtaaggcagcggtatcatcaacaggcttacccgtcttactgtcaagaggacatccggtcatgagcgcgcgttgacaattaatcatcggctcgtataatgcctctagaaataattcacacaggaaagtatacaatgagcaaaggagaagaacttttcactggagttgtcccaattcttgttgaattagatggtgatgttaatgggcacaaattttctgtccgtggagagggtgaaggtgatgctacaaacggaaaactcacccttaaatttatttgcactactggaaaactacctgttccgtggccaacacttgtcactactctgacctatggtgttcaatgcttttcccgttatccggatcacatgaaacggcatgactttttcaagagtgccatgcccgaaggttatgtacaggaacgcactatatctttcaaagatgacgggacctacaagacgcgtgctgaagtcaagtttgaaggtgatacccttgttaatcgtatcgagttaaagggtattgattttaaagaagatggaaacattcttggacacaaactcgagtacaactttaactcacacaatgtatacatcacggcagacaaacaaaagaatggaatcaaagctaacttcaaaattcgccacaacgttgaagatggttccgttcaactagcagaccattatcaacaaaatactccaattggcgatggccctgtccttttaccagacaaccattacctgtcgacacaatctgtcctttcgaaagatcccaacgaaaagcgtgaccacatggtccttcttgagtttgtaactgctgctgggattacacatggcatggatgagctctacaaataagatccggctgctaacaaagcccgaaaggaagctgagttggctgctgccaccgctgagcaataactagcataaccccttggggcctctaaacgg

SEQ ID NO: 7 - DNA, 4817 bp, synthetic construct
  source 1..4817: mol_type = other DNA
gtcttgaggggttttttgctgaaaggaggaactatatccggattggcgaatggggcgaattgggtaccgggccccccctcgagccgatcatattcaataacccttaatataacttcgtataatgtatgctatacgaagttattaggtctgaagaggagtttacgtcccatatggagtcccgcttaatcagcttgcttacgcaggaatgctgggatatccagataatccggctctttcgcagtttgcggcgcattgtcattcacgactttagcaaccggcttctgctcctgggtcagcggagccatcccgtgctgctggtagcgatccatcactggctgctgaacctgcttattagtcaccagagtgatttcaggacgtttgtccatgccgatacctgtcgcaacaacagttacgcgcagctcgtcattcatatccgggtcaagagaagtaccgataaccacggtcgcgttgtcggaagcaaatgcacggatggtgttacctaccgtttcgaactcatccagacgcaggtcgaagcccgctgtgatgtttaccagtacgccgcgtgcgccagacaggtcgatatcttccagcagcggagaagagatagccatttcagcagcttcttccgcacgatcttcaccgctcgccacaccagaacccatcattgcgtagcccatttcagacattacggtgcgtacgtctgcaaagtccacgttcatcaaacccggacgagtaatcagttcggcgataccttgcacagcgccttttagtacatcgttcgctgcgccaaacgcatccagcagggagataccacggcccagaactttcagcagtttgtcgttcgggatagtgatcagagagtccacatgcttggacagttcagtgatcccctgctccgcgaatgccatacgcttcttgccttcaaagttgaaaggcttagtgacgacagcaacggtcaggatacccaaatcttttgccacttcagcgacgactggtgctgcacctgtaccggtaccaccacccatacccgcagcaataaagaccatgtctgcaccttccagcgccgcacgcagtgcatcgcgatcctcatcagccgcattgcggccaacttctggattagcgccagcgcccagtcctttggtgataccgctaccgatttgaatcgtctgtccaaccgctgttttacgcagcgcttgtgcatcggtatttaccgcgaagaattcaacaccttcaatgcgctcacgcaccatgtgttcaacagcattaccgccgccgccgccgacgccgatgactttaatcaccgcgtcattggtaagttccattggttcaaacatagatcatcgacccctcattttattgccagatcagaagaactcgtcaagaaggcgatagaaggcgatgcgctgcgaatcgggagcggcgataccgtaaagcacgaggaagcggtcagcccattcgccgccaagctcttcagcaatatcacgggtagccaacgctatgtcctgatagcggtccgccacacccagccggccacagtcgatgaatccagaaaagcggccattttccaccatgatattcggcaagcaggcatcgccatgggtcacgacgagatcctcgccgtcgggcatgcgcgccttgagcctggcgaacagttcggccggcgcgagcccctgatgctcttcgtccagatcatcctgatcgacaagaccggcttccatccgagtacgtgctcgctcgatgcgatgtttcgcttggtggtcgaatgggcaggtagccggatcaagcgtatgcagccgccgcattgcatcagccatgatggatactttctcggcaggagcaaggtgagatgacaggagatcctgccccggcacttcgcccaatagcagccagtcccttcccgcttcagtgacaacgtcgagcacagctgcgcaaggaacgcccgtcgtggccagccacgatagccgcgctgcctcgtcctgcagttcattcagggcaccggacaggtcggtcttgacaaaaagaaccgggcgcccctgcgctgacagccggaacacggcggcatcagagcagccgattgtctgttgtgcccagtcatagccgaatagcctctccacccaagcggccggagaacctgcgtgcaatccatcttgttcaatcatgcgaaacgatcctcatcctgtctcttgatcagatcctgatcccctgcgccatcagatccttggcggcaagaaagccatccagtttactttgcagggcttcccaaccttaccagagggcgccccagctggcaattccactagaggacttcgattaggccaaataggccgttcagatccttccgtatttagccagtatgttctctagtgtggttcgttgtttttgcgtgagccatgagaacgaaccattgagatcatgcttactttgcatgtcactcaaaaattttgcctcaaaactggtgagctgaatttttgcagttaaagcatcgtgtagtgtttttcttagtccgttacgtaggtaggaatctgatgtaatggttgttggtattttgtcaccattcatttttatctggttgttctcaagttcggttacgagatccatttgtctatctagttcaacttggaaaatcaacgtatcagtcgggcggcctcgcttatcaaccaccaatttcatattgctgtaagtgtttaaatctttacttattggtttcaaaacccattggttaagccttttaaactcatggtagttattttcaagcattaacatgaacttaaattcatcaaggctaatctctatatttgccttgtgagttttcttttgtgttagttcttttaataaccactcataaatcctcatagagtatttgttttcaaaagacttaacatgttccagattatattttatgaatttttttaactggaaaagataaggcaatatctcttcactaaaaactaattctaatttttcgcttgagaacttggcatagtttgtccactggaaaatctcaaagcctttaaccaaaggattcctgatttccacagttctcgtcatcagctctctggttgctttagctaatacaccataagcattttccctactgatgttcatcatctgagcgtattggttataagtgaacgataccgtccgttctttccttgtagggttttcaatcgtggggttgagtagtgccacacagcataaaattagcttggtttcatgctccgttaagtcatagcgactaatcgctagttcatttgctttgaaaacaactaattcagacatacatctcaattggtctaggtgattttaatcactataccaattgagatgggctagtcaatgataattactagtccttttcctttgagttgtgggtatctgtaaattctgctagacctttgctggaaaacttgtaaattctgctagaccctctgtaaattccgctagacctttgtgtgttttttttgtttatattcaagtggttataatttatagaataaagaaagaataaaaaaagataaaaagaatagatcccagccctgtgtataactcactactttagtcagttccgcagtattacaaaaggatgtcgcaaacgctgtttgctcctctacaaaacagaccttaaaaccctaaaggcttaagtagcaccctcgcaagctcgggcaaatcgctgaatattccttttgtctccgaccatcaggcacctgagtcgctgtctttttcgtgacattcagttcgctgcgctcacggctctggcagtgaatgggggtaaatggcactacaggcgccttttatggattcatgcaaggaaactacccataatacaagaaaagcccgtcacgggcttctcagggcgttttatggcgggtctgctatgtggtgctatctgactttttgctgttcagcagttcctgccctctgattttccagtctgaccacttcggattatcccgtgacaggtcattcagactggctaatgcacccagtaaggcagcggtatcatcaacaggcttacccgtcttactgtcaagaggacatccggtcatgagcgcgcgttgacaattaatcatcggctcgtataatgcctctagaaataattcacacaggaaagtatacacatcatgaaatacctgctgccgaccgctgctgctggtctgctgctcctcgctgcccagccggcgatggccgatgatgatgatgatagcccgggtcagggtacgcagagcgaaaacagctgtacgcattttccgggtaacctgccgaatatgctgcgtgatctgcgtgatgcatttagccgtgtgaaaacattttttcagatgaaagatcagctggataatctgctgctgaaagaaagcctgctggaagattttaaaggttatctgggttgtcaggccctgagcgaaatgattcagttttatctggaagaagttatgccgcaggcagaaaatcaggatcctgatattaaagcacatgttaatagcctgggtgaaaatctgaaaacactgcgtctgcgtctgcgccgttgccatcgctttctgccgtgtgaaaataaaagcaaagcagtggaacaggttaaaaacgcatttaataaactgcaggaaaaaggtatctataaagccatgtcagaatttgatatctttatcaattatatcgaagcatatatgaccatgaaaatccgtaatcaccaccaccaccaccactgagatccggctgctaacaaagcccgaaaggctgctaacaaagcccgaaaggaagctgagttggctgctgccaccgctgagcaataactagcataaccccttggggcctctaaacgg

SEQ ID NO: 8 - DNA, 4802 bp, synthetic construct
  source 1..4802: mol_type = other DNA
gtcttgaggggttttttgctgaaaggaggaactatatccggattggcgaatggggcgaattgggtaccgggccccccctcgagccgatcatattcaataacccttaatataacttcgtataatgtatgctatacgaagttattaggtctgaagaggagtttacgtcccatatggagtcccgcttaatcagcttgcttacgcaggaatgctgggatatccagataatccggctctttcgcagtttgcggcgcattgtcattcacgactttagcaaccggcttctgctcctgggtcagcggagccatcccgtgctgctggtagcgatccatcactggctgctgaacctgcttattagtcaccagagtgatttcaggacgtttgtccatgccgatacctgtcgcaacaacagttacgcgcagctcgtcattcatatccgggtcaagagaagtaccgataaccacggtcgcgttgtcggaagcaaatgcacggatggtgttacctaccgtttcgaactcatccagacgcaggtcgaagcccgctgtgatgtttaccagtacgccgcgtgcgccagacaggtcgatatcttccagcagcggagaagagatagccatttcagcagcttcttccgcacgatcttcaccgctcgccacaccagaacccatcattgcgtagcccatttcagacattacggtgcgtacgtctgcaaagtccacgttcatcaaacccggacgagtaatcagttcggcgataccttgcacagcgccttttagtacatcgttcgctgcgccaaacgcatccagcagggagataccacggcccagaactttcagcagtttgtcgttcgggatagtgatcagagagtccacatgcttggacagttcagtgatcccctgctccgcgaatgccatacgcttcttgccttcaaagttgaaaggcttagtgacgacagcaacggtcaggatacccaaatcttttgccacttcagcgacgactggtgctgcacctgtaccggtaccaccacccatacccgcagcaataaagaccatgtctgcaccttccagcgccgcacgcagtgcatcgcgatcctcatcagccgcattgcggccaacttctggattagcgccagcgcccagtcctttggtgataccgctaccgatttgaatcgtctgtccaaccgctgttttacgcagcgcttgtgcatcggtatttaccgcgaagaattcaacaccttcaatgcgctcacgcaccatgtgttcaacagcattaccgccgccgccgccgacgccgatgactttaatcaccgcgtcattggtaagttccattggttcaaacatagatcatcgacccctcattttattgccagatcagaagaactcgtcaagaaggcgatagaaggcgatgcgctgcgaatcgggagcggcgataccgtaaagcacgaggaagcggtcagcccattcgccgccaagctcttcagcaatatcacgggtagccaacgctatgtcctgatagcggtccgccacacccagccggccacagtcgatgaatccagaaaagcggccattttccaccatgatattcggcaagcaggcatcgccatgggtcacgacgagatcctcgccgtcgggcatgcgcgccttgagcctggcgaacagttcggccggcgcgagcccctgatgctcttcgtccagatcatcctgatcgacaagaccggcttccatccgagtacgtgctcgctcgatgcgatgtttcgcttggtggtcgaatgggcaggtagccggatcaagcgtatgcagccgccgcattgcatcagccatgatggatactttctcggcaggagcaaggtgagatgacaggagatcctgccccggcacttcgcccaatagcagccagtcccttcccgcttcagtgacaacgtcgagcacagctgcgcaaggaacgcccgtcgtggccagccacgatagccgcgctgcctcgtcctgcagttcattcagggcaccggacaggtcggtcttgacaaaaagaaccgggcgcccctgcgctgacagccggaacacggcggcatcagagcagccgattgtctgttgtgcccagtcatagccgaatagcctctccacccaagcggccggagaacctgcgtgcaatccatcttgttcaatcatgcgaaacgatcctcatcctgtctcttgatcagatcctgatcccctgcgccatcagatccttggcggcaagaaagccatccagtttactttgcagggcttcccaaccttaccagagggcgccccagctggcaattccactagaggacttcgattaggccaaataggccgttcagatccttccgtatttagccagtatgttctctagtgtggttcgttgtttttgcgtgagccatgagaacgaaccattgagatcatgcttactttgcatgtcactcaaaaattttgcctcaaaactggtgagctgaatttttgcagttaaagcatcgtgtagtgtttttcttagtccgttacgtaggtaggaatctgatgtaatggttgttggtattttgtcaccattcatttttatctggttgttctcaagttcggttacgagatccatttgtctatctagttcaacttggaaaatcaacgtatcagtcgggcggcctcgcttatcaaccaccaatttcatattgctgtaagtgtttaaatctttacttattggtttcaaaacccattggttaagccttttaaactcatggtagttattttcaagcattaacatgaacttaaattcatcaaggctaatctctatatttgccttgtgagttttcttttgtgttagttcttttaataaccactcataaatcctcatagagtatttgttttcaaaagacttaacatgttccagattatattttatgaatttttttaactggaaaagataaggcaatatctcttcactaaaaactaattctaatttttcgcttgagaacttggcatagtttgtccactggaaaatctcaaagcctttaaccaaaggattcctgatttccacagttctcgtcatcagctctctggttgctttagctaatacaccataagcattttccctactgatgttcatcatctgagcgtattggttataagtgaacgataccgtccgttctttccttgtagggttttcaatcgtggggttgagtagtgccacacagcataaaattagcttggtttcatgctccgttaagtcatagcgactaatcgctagttcatttgctttgaaaacaactaattcagacatacatctcaattggtctaggtgattttaatcactataccaattgagatgggctagtcaatgataattactagtccttttcctttgagttgtgggtatctgtaaattctgctagacctttgctggaaaacttgtaaattctgctagaccctctgtaaattccgctagacctttgtgtgttttttttgtttatattcaagtggttataatttatagaataaagaaagaataaaaaaagataaaaagaatagatcccagccctgtgtataactcactactttagtcagttccgcagtattacaaaaggatgtcgcaaacgctgtttgctcctctacaaaacagaccttaaaaccctaaaggcttaagtagcaccctcgcaagctcgggcaaatcgctgaatattccttttgtctccgaccatcaggcacctgagtcgctgtctttttcgtgacattcagttcgctgcgctcacggctctggcagtgaatgggggtaaatggcactacaggcgccttttatggattcatgcaaggaaactacccataatacaagaaaagcccgtcacgggcttctcagggcgttttatggcgggtctgctatgtggtgctatctgactttttgctgttcagcagttcctgccctctgattttccagtctgaccacttcggattatcccgtgacaggtcattcagactggctaatgcacccagtaaggcagcggtatcatcaacaggcttacccgtcttactgtcaagaggacatccggtcatgagcgcgcgttgacaattaatcatcggctcgtataatgcctctagaaataattcacacaggaaagtatacacatcatgaaatacctgctgccgaccgctgctgctggtctgctgctcctcgctgcccagccggcgatggccagcccgggtcagggtacgcagagcgaaaacagctgtacgcattttccgggtaacctgccgaatatgctgcgtgatctgcgtgatgcatttagccgtgtgaaaacattttttcagatgaaagatcagctggataatctgctgctgaaagaaagcctgctggaagattttaaaggttatctgggttgtcaggccctgagcgaaatgattcagttttatctggaagaagttatgccgcaggcagaaaatcaggatcctgatattaaagcacatgttaatagcctgggtgaaaatctgaaaacactgcgtctgcgtctgcgccgttgccatcgctttctgccgtgtgaaaataaaagcaaagcagtggaacaggttaaaaacgcatttaataaactgcaggaaaaaggtatctataaagccatgtcagaatttgatatctttatcaattatatcgaagcatatatgaccatgaaaatccgtaatcaccaccaccaccaccactgagatccggctgctaacaaagcccgaaaggctgctaacaaagcccgaaaggaagctgagttggctgctgccaccgctgagcaataactagcataaccccttggggcctctaaacgg

SEQ ID NO: 9 - DNA, 600 bp, synthetic construct
  source 1..600: mol_type = other DNA
atgaaatacctgctgccgaccgctgctgctggtctgctgctcctcgctgcccagccggcgatggccgatgatgatgatgatagcccgggtcagggtacgcagagcgaaaacagctgtacgcattttccgggtaacctgccgaatatgctgcgtgatctgcgtgatgcatttagccgtgtgaaaacattttttcagatgaaagatcagctggataatctgctgctgaaagaaagcctgctggaagattttaaaggttatctgggttgtcaggccctgagcgaaatgattcagttttatctggaagaagttatgccgcaggcagaaaatcaggatcctgatattaaagcacatgttaatagcctgggtgaaaatctgaaaacactgcgtctgcgtctgcgccgttgccatcgctttctgccgtgtgaaaatggcggtggcagcggtggcaaaagcaaagcagtggaacaggttaaaaacgcatttaataaactgcaggaaaaaggtatctataaagccatgtcagaatttgatatctttatcaattatatcgaagcatatatgaccatgaaaatccgtaatcaccaccaccatcaccactaa

SEQ ID NO: 10 - DNA, 582 bp, synthetic construct
  source 1..582: mol_type = other DNA
atgaaatacctgctgccgaccgctgctgctggtctgctgctcctcgctgcccagccggcgatggccgatgatgatgatgatagcccgggtcagggtacgcagagcgaaaacagctgtacgcattttccgggttatctgccgaatatgctgcgtgatctgcgtgatgcatttagccgtgtgaaaacattttttcagatgaaagatcagctggataatctgctgctgaaagaaagcctgctggaagattttaaaggttatctgggttgtcaggccctgagcgaaatgattcagttttatctggaagaagttatgccgcaggcagaaaatcaggatcctgatattaaagcacatgttcagagcctgggtgaaaatctgaaagatctgcgtctgtggctgcgccgttgccatcgctttctgccgtgtgaaaataaaagcaaagcagtggaacaggttaaaaacgcatttaataaactgcaggaaaaaggtatctataaagccatgtcagaatttgatatctttatcaattatatcgaagcatatatgaccatgaaaatccgtaatcaccaccaccaccaccactag

SEQ ID NO: 11 - DNA, 579 bp, synthetic construct
  source 1..579: mol_type = other DNA
atgaaatacctgctgccgaccgctgctgctggtctgctgctcctcgctgcccagccggcgatggccgatgatgatgatgatagcccgggtcagggtacgcagagcgaaaacagctgtacgcattttccgggttatctgccgaatatgctgcgtgatctgcgtgatgcatttagccgtgtgaaaacattttttcagatgaaagatcagctggataatctgctgctgaaagaaagcctgctggaagattttaaaggttatctgggttgtcaggccctgagcgaaatgattcagttttatctggaagaagttatgccgcaggcagaaaatcaggatcctgatattaaagcacatgttcagagcctgggtgaaaatctgaaagatctgcgtctgtggctgcgccgttgccatcgctttctgccgtgtgaaaatggcggtggcagcggtggcaaaagcaaagcagtggaacaggttaaaaacgcatttaataaactgcaggaaaaaggtatctataaagccatgtcagaatttgatatctttatcaattatatcgaagcatatatgaccatgaaaatccgtaat

SEQ ID NO: 12 - protein, 160 aa, synthetic construct
SPGQGTQSENSCTHFPGNLPNMLRDLRDAFSRVKTFFQMKDQLDNLLLKESLLEDFKGYLGCQALSEMIQFYLEEVMPQAENQDPDIKAHVNSLGENLKTLRLRLRRCHRFLPCENKSKAVEQVKNAFNKLQEKGIYKAMSEFDIFINYIEAYMTMKIRN

SEQ ID NO: 13 - protein, 166 aa, synthetic construct
SPGQGTQSENSCTHFPGNLPNMLRDLRDAFSRVKTFFQMKDQLDNLLLKESLLEDFKGYLGCQALSEMIQFYLEEVMPQAENQDPDIKAHVNSLGENLKTLRLRLRRCHRFLPCENGGGSGGKSKAVEQVKNAFNKLQEKGIYKAMSEFDIFINYIEAYMTMKIRN

SEQ ID NO: 14 - protein, 160 aa, synthetic construct
SPGQGTQSENSCTHFPGYLPNMLRDLRDAFSRVKTFFQMKDQLDNLLLKESLLEDFKGYLGCQALSEMIQFYLEEVMPQAENQDPDIKAHVQSLGENLKDLRLWLRRCHRFLPCENKSKAVEQVKNAFNKLQEKGIYKAMSEFDIFINYIEAYMTMKIRN

SEQ ID NO: 15 - protein, 166 aa, synthetic construct
SPGQGTQSENSCTHFPGYLPNMLRDLRDAFSRVKTFFQMKDQLDNLLLKESLLEDFKGYLGCQALSEMIQFYLEEVMPQAENQDPDIKAHVQSLGENLKDLRLWLRRCHRFLPCENGGGSGGKSKAVEQVKNAFNKLQEKGIYKAMSEFDIFINYIEAYMTMKIRN

SEQ ID NO: 16 - protein, 22 aa, synthetic construct
MKYLLPTAAAGLLLLAAQPAMA

SEQ ID NO: 17 - protein, 187 aa, synthetic construct
MKYLLPTAAAGLLLLAAQPAMADDDDDSPGQGTQSENSCTHFPGNLPNMLRDLRDAFSRVKTFFQMKDQLDNLLLKESLLEDFKGYLGCQALSEMIQFYLEEVMPQAENQDPDIKAHVNSLGENLKTLRLRLRRCHRFLPCENKSKAVEQVKNAFNKLQEKGIYKAMSEFDIFINYIEAYMTMKIRN

SEQ ID NO: 18 - protein, 193 aa, synthetic construct
MKYLLPTAAAGLLLLAAQPAMADDDDDSPGQGTQSENSCTHFPGNLPNMLRDLRDAFSRVKTFFQMKDQLDNLLLKESLLEDFKGYLGCQALSEMIQFYLEEVMPQAENQDPDIKAHVNSLGENLKTLRLRLRRCHRFLPCENGGGSGGKSKAVEQVKNAFNKLQEKGIYKAMSEFDIFINYIEAYMTMKIRN

SEQ ID NO: 19 - protein, 187 aa, synthetic construct
MKYLLPTAAAGLLLLAAQPAMADDDDDSPGQGTQSENSCTHFPGYLPNMLRDLRDAFSRVKTFFQMKDQLDNLLLKESLLEDFKGYLGCQALSEMIQFYLEEVMPQAENQDPDIKAHVQSLGENLKDLRLWLRRCHRFLPCENKSKAVEQVKNAFNKLQEKGIYKAMSEFDIFINYIEAYMTMKIRN

SEQ ID NO: 20 - protein, 193 aa, synthetic construct
MKYLLPTAAAGLLLLAAQPAMADDDDDSPGQGTQSENSCTHFPGYLPNMLRDLRDAFSRVKTFFQMKDQLDNLLLKESLLEDFKGYLGCQALSEMIQFYLEEVMPQAENQDPDIKAHVQSLGENLKDLRLWLRRCHRFLPCENGGGSGGKSKAVEQVKNAFNKLQEKGIYKAMSEFDIFINYIEAYMTMKIRN

SEQ ID NO: 21 - protein, 186 aa, synthetic construct
MKYLLPTAAAGLLLLAAQPAMADDDDSPGQGTQSENSCTHFPGNLPNMLRDLRDAFSRVKTFFQMKDQLDNLLLKESLLEDFKGYLGCQALSEMIQFYLEEVMPQAENQDPDIKAHVNSLGENLKTLRLRLRRCHRFLPCENKSKAVEQVKNAFNKLQEKGIYKAMSEFDIFINYIEAYMTMKIRN

SEQ ID NO: 22 - protein, 192 aa, synthetic construct
MKYLLPTAAAGLLLLAAQPAMADDDDSPGQGTQSENSCTHFPGNLPNMLRDLRDAFSRVKTFFQMKDQLDNLLLKESLLEDFKGYLGCQALSEMIQFYLEEVMPQAENQDPDIKAHVNSLGENLKTLRLRLRRCHRFLPCENGGGSGGKSKAVEQVKNAFNKLQEKGIYKAMSEFDIFINYIEAYMTMKIRN

SEQ ID NO: 23 - protein, 186 aa, synthetic construct
MKYLLPTAAAGLLLLAAQPAMADDDDSPGQGTQSENSCTHFPGYLPNMLRDLRDAFSRVKTFFQMKDQLDNLLLKESLLEDFKGYLGCQALSEMIQFYLEEVMPQAENQDPDIKAHVQSLGENLKDLRLWLRRCHRFLPCENKSKAVEQVKNAFNKLQEKGIYKAMSEFDIFINYIEAYMTMKIRN

SEQ ID NO: 24 - protein, 192 aa, synthetic construct
MKYLLPTAAAGLLLLAAQPAMADDDDSPGQGTQSENSCTHFPGYLPNMLRDLRDAFSRVKTFFQMKDQLDNLLLKESLLEDFKGYLGCQALSEMIQFYLEEVMPQAENQDPDIKAHVQSLGENLKDLRLWLRRCHRFLPCENGGGSGGKSKAVEQVKNAFNKLQEKGIYKAMSEFDIFINYIEAYMTMKIRN

SEQ ID NO: 25 - DNA, 85 bp, synthetic construct
  source 1..85: mol_type = other DNA
gcaggggtaaaagtgacctgacgcaatatttgtcttttcttgcttcttaataatgttgtcacaaaaagtgagggtgactacatgg

SEQ ID NO: 26 - DNA, 85 bp, synthetic construct
  source 1..85: mol_type = other DNA
cgccgcaaagtttgagcgaagtcaataaactctctacccattcagggcaatatctctcttgcaggtgaatgcaacgtcaagcgat

SEQ ID NO: 27 - DNA, 85 bp, synthetic construct
  source 1..85: mol_type = other DNA
tcagaagaagcaaaaagacactttaccgaagggtttaacattttttcgtgatactcatcaccatgacgcaaatgcgttgcataaa

SEQ ID NO: 28 - DNA, 85 bp, synthetic construct
  source 1..85: mol_type = other DNA
aaccgaggtcacaacatagtaaaagcgctattggtaatggtacaatcgcgcgtttacacttattcagaacgatttttttcaggag

SEQ ID NO: 29 - DNA, 54 bp, synthetic construct
  source 1..54: mol_type = other DNA
ggataaaagtgacctgacgcaatatttgtcttttcttgcttaataatgttgtca

SEQ ID NO: 30 - DNA, 35 bp, synthetic construct
  source 1..35: mol_type = other DNA
tgtaagtttatacataggcgagtactctgttatgg

SEQ ID NO: 31 - DNA, 74 bp, synthetic construct
  source 1..74: mol_type = other DNA
ttaaatttcctctcgtcaggccggaataactccctataatgcgccaccacactgatagtgctagtgtagatcac

SEQ ID NO: 32 - DNA, 58 bp, synthetic construct
  source 1..58: mol_type = other DNA
aaaattgatctgaatcaatattttgacaaaaattgatctgaatcaatatttactgagc

SEQ ID NO: 33 - DNA, 44 bp, synthetic construct
  source 1..44: mol_type = other DNA
gttaataaaatgttattgacagttaataaaatgttatactgagc

SEQ ID NO: 34 - DNA, 30 bp, synthetic construct
  source 1..30: mol_type = other DNA
ttagcacgttaattatctatcgtgtatatg

SEQ ID NO: 35 - DNA, 27 bp, synthetic construct
  source 1..27: mol_type = other DNA
caccaccaccaccaccactgagatccg

SEQ ID NO: 36 - DNA, 33 bp, synthetic construct
  source 1..33: mol_type = other DNA
atcatcatcatcatcggccatcgccggctgggc

SEQ ID NO: 37 - DNA, 40 bp, synthetic construct
  source 1..40: mol_type = other DNA
tggccgatgatgatgatgatagcccgggtcagggtacgca

SEQ ID NO: 38 - DNA, 48 bp, synthetic construct
  source 1..48: mol_type = other DNA
tcagtggtggtggtggtggtgattacggattttcatggtcatatatgc

SEQ ID NO: 39 - DNA, 25 bp, synthetic construct
  source 1..25: mol_type = other DNA
tggccagcccgggtcagggtacgca

SEQ ID NO: 40 - DNA, 48 bp, synthetic construct; identical to SEQ ID NO: 38
  source 1..48: mol_type = other DNA

SEQ ID NO: 41 - DNA, 19 bp, synthetic construct
  source 1..19: mol_type = other DNA
ctcgacgctctcccttatg

SEQ ID NO: 42 - DNA, 23 bp, synthetic construct
  source 1..23: mol_type = other DNA
ctgacatggctttatagatacct

SEQ ID NO: 43 - DNA, 20 bp, synthetic construct
  source 1..20: mol_type = other DNA
ctgctaacaaagcccgaaag

SEQ ID NO: 44 - DNA, 27 bp, synthetic construct
  source 1..27: mol_type = other DNA
ctttcctgtgtgaattatttctagagg

SEQ ID NO: 45 - DNA, 48 bp, synthetic construct
  source 1..48: mol_type = other DNA
aaataattcacacaggaaagtatacacatcatgaaatacctgctgccg

SEQ ID NO: 46 - DNA, 40 bp, synthetic construct
  source 1..40: mol_type = other DNA
ctttcgggctttgttagcagcctttcgggctttgttagca

SEQ ID NO: 47 - DNA, 21 bp, synthetic construct
  source 1..21: mol_type = other DNA
ccgtcttactgtcaagaggac

SEQ ID NO: 48 - DNA, 23 bp, synthetic construct
  source 1..23: mol_type = other DNA
ctgacatggctttatagatacct

SEQ ID NO: 49 - DNA, 20 bp, synthetic construct
  source 1..20: mol_type = other DNA
caccgctgagcaataactag

SEQ ID NO: 50 - DNA, 1923 bp, synthetic construct
  source 1..1923: mol_type = other DNA
ccaccgctgagcaataactagcataaccccttggggcctctaaacgggtcttgaggggttttttgctgaaaggaggaactatatccggattggcgaatgggtcagaagaactcgtcaagaaggcgatagaaggcgatgcgctgcgaatcgggagcggcgataccgtaaagcacgaggaagcggtcagcccattcgccgccaagctcttcagcaatatcacgggtagccaacgctatgtcctgatagcggtccgccacacccagccggccacagtcgatgaatccagaaaagcggccattttccaccatgatattcggcaagcaggcatcgccatgggtcacgacgagatcctcgccgtcgggcatgcgcgccttgagcctggcgaacagttcggccggcgcgagcccctgatgctcttcgtccagatcatcctgatcgacaagaccggcttccatccgagtacgtgctcgctcgatgcgatgtttcgcttggtggtcgaatgggcaggtagccggatcaagcgtatgcagccgccgcattgcatcagccatgatggatactttctcggcaggagcaaggtgagatgacaggagatcctgccccggcacttcgcccaatagcagccagtcccttcccgcttcagtgacaacgtcgagcacagctgcgcaaggaacgcccgtcgtggccagccacgatagccgcgctgcctcgtcctgcagttcattcagggcaccggacaggtcggtcttgacaaaaagaaccgggcgcccctgcgctgacagccggaacacggcggcatcagagcagccgattgtctgttgtgcccagtcatagccgaatagcctctccacccaagcggccggagaacctgcgtgcaatccatcttgttcaatcatgcgaaacgatcctcatcctgtctcttgatcagatcctgatcccctgcgccatcagatccttggcggcaagaaagccatccagtttactttgcagggcttcccaaccttaccagagggcgccccagctggcaattccactagaggacttcgattaggccaaatagcctttttgataatctcatgaccaaaatcccttaacgtgagttttcgttccactgagcgtcagaccccgtagaaaagatcaaaggatcttcttgagatcctttttttctgcgcgtaatctgctgcttgcaaacaaaaaaaccaccgctaccagcggtggtttgtttgccggatcaagagctaccaactctttttccgaaggtaactggcttcagcagagcgcagataccaaatactgttcttctagtgtagccgtagttaggccaccacttcaagaactctgtagcaccgcctacatacctcgctctgctaatcctgttaccagtggctgctgccagtggcgataagtcgtgtcttaccgggttggactcaagacgatagttaccggataaggcgcagcggtcgggctgaacggggggttcgtgcacacagcccagcttggagcgaacgacctacaccgaactgagatacctacagcgtgagctatgagaaagcgccacgcttcccgaagggagaaaggcggacaggtatccggtaagcggcagggtcggaacaggagagcgcacgagggagcttccagggggaaacgcctggtatctttatagtcctgtcgggtttcgccacctctgacttgagcgtcgatttttgtgatgctcgtcaggggggcggagcctatggaaaaacgccagcaacgcggcctttttacggttcctggccttttgctggccttttgctcacatgttctttcctgcgttatcccctgattctgtggacaagaggacatccggtcatgagcgcgcgttgacaattaatcatcggctcgtataatgcctctagaaataattcacacaggaaagtatacaca

SEQ ID NO: 51 - DNA, 2574 bp, synthetic construct
  source 1..2574: mol_type = other DNA
gtgtgaaaacattttttcagatgaaagatcagctggataatctgctgctgaaagaaagcctgctggaagattttaaaggttatctgggttgtcaggccctgagcgaaatgattcagttttatctggaagaagttatgccgcaggcagaaaatcaggatcctgatattaaagcacatgttaatagcctgggtgaaaatctgaaaacactgcgtctgcgtctgcgccgttgccatcgctttctgccgtgtgaaaataaaagcaaagcagtggaacaggttaaaaacgcatttaataaactgcaggaaaaaggtatctataaagccatgtcagaatttgatatctttatcaattatatcgaagcatatatgaccatgaaaatccgtaatcaccaccaccaccaccactgagatccggctgctaacaaagcccgaaaggctgctaacaaagcccgaaaggaagctgagttggctgctgccaccgctgagcaataactagcataaccccttggggcctctaaacgggtcttgaggggttttttgctgaaaggaggaactatatccggattggcgaatgggtcagaagaactcgtcaagaaggcgatagaaggcgatgcgctgcgaatcgggagcggcgataccgtaaagcacgaggaagcggtcagcccattcgccgccaagctcttcagcaatatcacgggtagccaacgctatgtcctgatagcggtccgccacacccagccggccacagtcgatgaatccagaaaagcggccattttccaccatgatattcggcaagcaggcatcgccatgggtcacgacgagatcctcgccgtcgggcatgcgcgccttgagcctggcgaacagttcggccggcgcgagcccctgatgctcttcgtccagatcatcctgatcgacaagaccggcttccatccgagtacgtgctcgctcgatgcgatgtttcgcttggtggtcgaatgggcaggtagccggatcaagcgtatgcagccgccgcattgcatcagccatgatggatactttctcggcaggagcaaggtgagatgacaggagatcctgccccggcacttcgcccaatagcagccagtcccttcccgcttcagtgacaacgtcgagcacagctgcgcaaggaacgcccgtcgtggccagccacgatagccgcgctgcctcgtcctgcagttcattcagggcaccggacaggtcggtcttgacaaaaagaaccgggcgcccctgcgctgacagccggaacacggcggcatcagagcagccgattgtctgttgtgcccagtcatagccgaatagcctctccacccaagcggccggagaacctgcgtgcaatccatcttgttcaatcatgcgaaacgatcctcatcctgtctcttgatcagatcctgatcccctgcgccatcagatccttggcggcaagaaagccatccagtttactttgcagggcttcccaaccttaccagagggcgccccagctggcaattccactagaggacttcgattaggccaaatagcctttttgataatctcatgaccaaaatcccttaacgtgagttttcgttccactgagcgtcagaccccgtagaaaagatcaaaggatcttcttgagatcctttttttctgcgcgtaatctgctgcttgcaaacaaaaaaaccaccgctaccagcggtggtttgtttgccggatcaagagctaccaactctttttccgaaggtaactggcttcagcagagcgcagataccaaatactgttcttctagtgtagccgtagttaggccaccacttcaagaactctgtagcaccgcctacatacctcgctctgctaatcctgttaccagtggctgctgccagtggcgataagtcgtgtcttaccgggttggactcaagacgatagttaccggataaggcgcagcggtcgggctgaacggggggttcgtgcacacagcccagcttggagcgaacgacctacaccgaactgagatacctacagcgtgagctatgagaaagcgccacgcttcccgaagggagaaaggcggacaggtatccggtaagcggcagggtcggaacaggagagcgcacgagggagcttccagggggaaacgcctggtatctttatagtcctgtcgggtttcgccacctctgacttgagcgtcgatttttgtgatgctcgtcaggggggcggagcctatggaaaaacgccagcaacgcggcctttttacggttcctggccttttgctggccttttgctcacatgttctttcctgcgttatcccctgattctgtggacaagaggacatccggtcatgagcgcgcgttgacaattaatcatcggctcgtataatgcctctagaaataattcacacaggaaagtatacacatcatgaaatacctgctgccgaccgctgctgctggtctgctgctcctcgctgcccagccggcgatggccgatgatgatgatgatagcccgggtcagggtacgcagagcgaaaacagctgtacgcattttccgggtaacctgccgaatatgctgcgtgatctgcgtgatgcatttagcc

SEQ ID NO: 52 - DNA, 2574 bp, synthetic construct
  source 1..2574: mol_type = other DNA
caccaccaccaccaccactgagatccggctgctaacaaagcccgaaaggctgctaacaaagcccgaaaggaagctgagttggctgctgccaccgctgagcaataactagcataaccccttggggcctctaaacgggtcttgaggggttttttgctgaaaggaggaactatatccggattggcgaatgggtcagaagaactcgtcaagaaggcgatagaaggcgatgcgctgcgaatcgggagcggcgataccgtaaagcacgaggaagcggtcagcccattcgccgccaagctcttcagcaatatcacgggtagccaacgctatgtcctgatagcggtccgccacacccagccggccacagtcgatgaatccagaaaagcggccattttccaccatgatattcggcaagcaggcatcgccatgggtcacgacgagatcctcgccgtcgggcatgcgcgccttgagcctggcgaacagttcggccggcgcgagcccctgatgctcttcgtccagatcatcctgatcgacaagaccggcttccatccgagtacgtgctcgctcgatgcgatgtttcgcttggtggtcgaatgggcaggtagccggatcaagcgtatgcagccgccgcattgcatcagccatgatggatactttctcggcaggagcaaggtgagatgacaggagatcctgccccggcacttcgcccaatagcagccagtcccttcccgcttcagtgacaacgtcgagcacagctgcgcaaggaacgcccgtcgtggccagccacgatagccgcgctgcctcgtcctgcagttcattcagggcaccggacaggtcggtcttgacaaaaagaaccgggcgcccctgcgctgacagccggaacacggcggcatcagagcagccgattgtctgttgtgcccagtcatagccgaatagcctctccacccaagcggccggagaacctgcgtgcaatccatcttgttcaatcatgcgaaacgatcctcatcctgtctcttgatcagatcctgatcccctgcgccatcagatccttggcggcaagaaagccatccagtttactttgcagggcttcccaaccttaccagagggcgccccagctggcaattccactagaggacttcgattaggccaaatagcctttttgataatctcatgaccaaaatcccttaacgtgagttttcgttccactgagcgtcagaccccgtagaaaagatcaaaggatcttcttgagatcctttttttctgcgcgtaatctgctgcttgcaaacaaaaaaaccaccgctaccagcggtggtttgtttgccggatcaagagctaccaactctttttccgaaggtaactggcttcagcagagcgcagataccaaatactgttcttctagtgtagccgtagttaggccaccacttcaagaactctgtagcaccgcctacatacctcgctctgctaatcctgttaccagtggctgctgccagtggcgataagtcgtgtcttaccgggttggactcaagacgatagttaccggataaggcgcagcggtcgggctgaacggggggttcgtgcacacagcccagcttggagcgaacgacctacaccgaactgagatacctacagcgtgagctatgagaaagcgccacgcttcccgaagggagaaaggcggacaggtatccggtaagcggcagggtcggaacaggagagcgcacgagggagcttccagggggaaacgcctggtatctttatagtcctgtcgggtttcgccacctctgacttgagcgtcgatttttgtgatgctcgtcaggggggcggagcctatggaaaaacgccagcaacgcggcctttttacggttcctggccttttgctggccttttgctcacatgttctttcctgcgttatcccctgattctgtggacaagaggacatccggtcatgagcgcgcgttgacaattaatcatcggctcgtataatgcctctagaaataattcacacaggaaagtatacacatcatgaaatacctgctgccgaccgctgctgctggtctgctgctcctcgctgcccagccggcgatggccgatgatgatgatgatagccgcggccagtacagccgcgaggacaataactgcacccattttccggtgggccagagccatatgctgctggaactgcgcaccgcgtttagccaagttaagacgttcttccagaccaaagaccagctggataacattttactgaccgactctttaatgcaagattttaagggctatctgggctgccaagctttaagcgagatgatccagttctatttagtggaagtgatgccgcaagctgaaaaacacggcccggagatcaaagaacatttaaactctttaggcgagaaactgaagactttacgcatgcgtttacgtcgttgccatcgctttctgccgtgcgagaacaaaagcaaagcggtggagcaagttaagagcgacttcaacaaactgcaagatcaaggtgtgtataaggcgatgaacgaattcgatatctttatcaactgcatcgaagcgtatatgatgattaaaatgaaaagc

SEQ ID NO: 53 - DNA, 3977 bp, synthetic construct
  source 1..3977: mol_type = other DNA
ttcacagaaaagtgttgcccccttccatggcggaagggggacaaaggtgaatttgtcctactcaggagagcgttcaccgacaaacaacagataaaacgaaaggcccagtctttcgactgagcctttcgttttatttgatgcactagtgccgatcatattcaataacccttaatataacttcgtataatgtatgctatacgaagttattaggtctgaagaggagtttacgtcccatatggagtcccgctcagaagaactcgtcaagaaggcgatagaaggcgatgcgctgcgaatcgggagcggcgataccgtaaagcacgaggaagcggtcagcccattcgccgccaagctcttcagcaatatcacgggtagccaacgctatgtcctgatagcggtccgccacacccagccggccacagtcgatgaatccagaaaagcggccattttccaccatgatattcggcaagcaggcatcgccatgggtcacgacgagatcctcgccgtcgggcatgcgcgccttgagcctggcgaacagttcggccggcgcgagcccctgatgctcttcgtccagatcatcctgatcgacaagaccggcttccatccgagtacgtgctcgctcgatgcgatgtttcgcttggtggtcgaatgggcaggtagccggatcaagcgtatgcagccgccgcattgcatcagccatgatggatactttctcggcaggagcaaggtgagatgacaggagatcctgccccggcacttcgcccaatagcagccagtcccttcccgcttcagtgacaacgtcgagcacagctgcgcaaggaacgcccgtcgtggccagccacgatagccgcgctgcctcgtcctgcagttcattcagggcaccggacaggtcggtcttgacaaaaagaaccgggcgcccctgcgctgacagccggaacacggcggcatcagagcagccgattgtctgttgtgcccagtcatagccgaatagcctctccacccaagcggccggagaacctgcgtgcaatccatcttgttcaatcatgcgaaacgatcctcatcctgtctcttgatcagatcctgatcccctgcgccatcagatccttggcggcaagaaagccatccagtttactttgcagggcttcccaaccttaccagagggcgccccagctggcaattccgacgtcattgcgttgctagccaagcttaggatccggaacccttaatataacttcgtataatgtatgctatacgaagttattaggtccctcgaagaggttcactagctatctagagcttggactcctgttgatagatccagtaatgacctcagaactccatctggatttgttcagaacgctcggttgccgccgggcgttttttattggtgagaatccaagcccgggaaacgggatcctgatcttgatcaggctgtgggtcaggccactcttggcatcgacaccaatgtgggccttcatgccaaagtgccactgattgcctttcttggtctgatgcatctccggatcgcgttgctgctctttgttcttggtcgagctgggtgcctcaatgatggtggcatcgaccaaggtgccttgagtcatcatgacgcctgcttcggccagccagcgattgatggtcttgaacaattggcgggccagttgatgctgctccagcaggtggcggaaattcatgatggtggtgcggtccggcaaggcgctatccagggataaccgggcaaacagacgcatggaggcgatttcgtacagagcatcttccatcgcgccatcgctcaggttgtaccaatgctgcatgcagtgaatgcgtagcatggtttccagcggataaggtcgccggccattaccagccttggggtaaaacggctcgatgacttccaccatgttttgccatggcagaatctgctccatgcgggacaagaaaatctcttttctggtctgacggcgcttactgctgaattcactgtcggcgaaggtaagttgatgactcatgatgaaccctgttctatggctccagatgacaaacatgatctcatatcagggacttgttcgcaccttccttagcacgttaattatctatcgtgtatatggaggggatctagaatgaaaaaaataatgctagtttttattacacttatattagttagtctaccaattgcgcaacaaactgaagcaaaggatgcatctgcattcaataaagaaaattcaatttcatccatggcaccaccagcatctccgcctgcaagtcctaagacgccaatcgaaaagaaacacgcggatgaaatcgataagtatatacaaggattggactacaataaaaacaatgtattagtataccacggagatgcagtgacaaatgtgccgccaagaaaaggttacaaagatggaaatgaatatattgttgtggagaaaaagaagaaatccatcaatcaaaataatgcagacattcaagttgtgaatgcaatttcgagcctaacctatccaggtgctctcgtaaaagcgaattcggaattagtagaaaatcaaccagatgttctccctgtaaaacgtgattcattaacactcagcattgatttgccaggtatgactaatcaagacaataaaatcgttgtaaaaaatgccactaaatcaaacgttaacaacgcagtaaatacattagtggaaagatggaatgaaaaatatgctcaagcttatccaaatgtaagtgcaaaaattgattatgatgacgaaatggcttacagtgaatcacaattaattgcgaaatttggtacagcatttaaagctgtaaataatagcttgaatgtaaacttcggcgcaatcagtgaagggaaaatgcaagaagaagtcattagttttaaacaaatttactataacgtgaatgttaatgaacctacaagaccttccagatttttcggcaaagctgttactaaagagcagttgcaagcgcttggagtgaatgcagaaaatcctcctgcatatatctcaagtgtggcgtatggccgtcaagtttatttgaaattatcaactaattcccatagtactaaagtaaaagctgcttttgatgctgccgtaagcggaaaatctgtctcaggtgatgtagaactaacaaatatcatcaaaaattcttccttcaaagccgtaatttacggaggttccgcaaaagatgaagttcaaatcatcgacggcaacctcggagacttacgagatattttgaaaaaaggcgctacttttaatcgagaaacaccaggagttcccattgcttatacaacaaacttcctaaaagacaatgaattagctgttattaaaaacaactcagaatatattgaaacaacttcaaaagcttatacagatggaaaaattaacatcgatcactctggaggatacgttgctcaattcaacatttcttgggatgaagtaaattatgatcctgaaggtaacgaaattgttcaacataaaaactggagcgaaaacaataaaagtaagctagctcatttcacatcgtccatctatttgccaggtaacgcgagaaatattaatgtttacgctaaagaatgcactggtttagcttgggaatggtggagaacggtaattgatgaccggaacttaccacttgtgaaaaatagaaatatctccatctggggcaccacgctttatccgaaatatagtaataaagtagataatccaatcgaataagtcgacctcgaggactagtgaacctcttcgagggacctaataacttcgtatagcatacattatacgaagttatattaagggttattgaatatgatcggctcgagattacttcgcattgcaatcagctacggactcaagcttacgtcaggtcatacgatgaaggcgataagtcgcgtaagttgctagcccacgcggctcaccttcacgggtgggcctttcttcggtgtttcaatctcgattaacaggtaacgcaaaattgctgtgtacgtcaga

SEQ ID NO: 54 - DNA, 2716 bp, synthetic construct
  source 1..2716: mol_type = other DNA
ttggtttcagtgaatcccgttatcagcagttttttgatgaggtgtagtctatttgtcctactcaggagagcgttcaccgacaaacaacagataaaacgaaaggcccagtctttcgactgagcctttcgttttatttgatgcactagtgccgatcatattcaataacccttaatataacttcgtataatgtatgctatacgaagttattaggtctgaagaggagtttacgtcccatatggagtcccgcttacgccccgccctgccactcatcgcagtactgttgtaattcattaagcattctgccgacatggaagccatcacagacggcatgatgaacctgaatcgccagcggcatcagcaccttgtcgccttgcgtataatatttgcccatggtgaaaacgggggcgaagaagttgtccatattggccacgtttaaatcaaaactggtgaaactcacccagggattggctgagacgaaaaacatattctcaataaaccctttagggaaataggccaggttttcaccgtaacacgccacatcttgcgaatatatgtgtagaaactgccggaaatcgtcgtggtattcactccagagcgatgaaaacgtttcagtttgctcatggaaaacggtgtaacaagggtgaacactatcccatatcaccagctcaccgtctttcattgccatacgaaattccggatgagcattcatcaggcgggcaagaatgtgaataaaggccggataaaacttgtgcttatttttctttacggtctttaaaaaggccgtaatatccagctgaacggtctggttataggtacattgagcaactgactgaaatgcctcaaaatgttctttacgatgccattgggatatatcaacggtggtatatccagtgatttttttctccatgcgaaacgatcctcatcctgtctcttgatcagatcctgatcccctgcgccatcagatccttggcggcaagaaagccatccagtttactttgcagggcttcccaaccttaccagagggcgccccagctggcaattccgacgtcattgcgttgctagccaagcttaggatccggaacccttaatataacttcgtataatgtatgctatacgaagttattaggtccctcgaagaggttcactagctatctagagcttggactcctgttgatagatccagtaatgacctcagaactccatctggatttgttcagaacgctcggttgccgccgggcgttttttattggtgagaatccaagcccgggaaacgggatcctgatcttgatcaaccgaggtcacaacatagtaaaagcgctattggtaatggtacaatcgcgcgtttacacttattcagaacgatttttttcaggagggcctacttgtcacacaggacggtaatgtcgtgcccggttattgagctgacacagcaacttattcgtcgcccctccctgagtccggatgacgcaggctgtcaggcattaatgattgaacgcctgcgtaaaatcggttttaccattgagcatatggattttggcgacacgcaaaatttttgggcatggcgtgggcgtggcgaaacgctggcgttcgccgggcatactgacgtcgtaccggctggcgatgtcgatcgctggatcaatccgccgtttgagcctacgattcgcgacggaatgttgttcggtcgcggcgcggcggatatgaaaggttcactggcggccatggtggtggctgctgaacgttttgttgcgcagcatcctcatcaccggggccgcctcgcatttttgattacctctgatgaggaagccagcgcaaaaaatggcaccgtaaaggtggttgaagcgctgatggcccgtaacgagcggctggattactgtctggtcggcgaaccttccagtactgaaattgtgggcgatgtcgtcaaaaacgggcgtcgcggttctctcacctgtaacctcactatccatggcgttcaggggcacgtcgcctatccgcatctggcggataaccctgttcatcgcgccgcgccttttcttaatgaactggtcgctatcgagtgggatcggggcaatgactttttcccggccaccagtatgcaggtagccaatatccaggcaggcaccggcagcaataatgtcattcccggcgaactgttcgtgcagtttaacttccgtttcagcacggaactgaccgatgagatgatcaaagagcgggtacatgcgctgcttgaaaagcatcagctacgctataccgtagactggtggctttccgggcagccgttcctgaccgcacgcggcaagctggtggacgcggtggtaaacgccattgagcactataatgaaattaaaccgcaattactgacgacgggcggtacgtccgacggacgttttatcgcccgtatgggagcgcaggtggtagaactggggccggtgaacgccaccattcataaaattaatgaatgtgtgaatgccgccgatctccagctactggcccgtatgtatcaacgcattatggaacagctcgtcgcccatcaccatcaccatcactaagattacttcgcattgcaatcagctacggactcaagcttacgtcaggtcatacgatgaaggcgataagtcgcgtaagttgctagcccacgcggctcaccttcacgggtgggcctttcttcgtgagcgttccggtaagaggaaataagcatggactggctggcaaaatattg

SEQ ID NO: 55 - DNA, 6750 bp, synthetic construct
  source 1..6750: mol_type = other DNA
catggtcatagctgtttcctttaatgcccatggcgtttaccaatgcttaatcagtgaggcacctatctcagcgatctgtctatttcgttcatccatagttgcctgactccccgtcgtgtagataactacgatacgggagggcttaccatctggccccagtgctgcaatgataccgcgacttccacgctcaccggctccagatttatcagcaataaaccagccagccggaagggccgagcgcagaagtggtcctgcaactttatccgcctccatccagtctattaattgttgccgggaagctagagtaagtagttcgccagttaatagtttgcgcaacgttgttgccattgctacaggcatcgtggtgtcacgctcgtcgtttggtatggcttcattcagctccggttcccaacgatcaaggcgagttacatgatcccccatgttgtgcaaaaaagcggttagctccttcggtcctccgatcgttgtcagaagtaagttggccgcagtgttatcactcatggttatggcagcactgcataattctcttactgtcatgccatccgtaagatgcttttctgtgactggtgagtactcaaccaagtcattctgagaatagtgtatgcggcgaccgagttgctcttgcccggcgtcaatacgggataataccgcgccacatagcagaactttaaaagtgctcatcattggaaaacgttcttcggggcgaaaactctcaaggatcttaccgctgttgagatccagttcgatgtaacccactcgtgcacccaactgatcttcagcatcttttactttcaccagcgtttctgggtgagcaaaaacaggaaggcaaaatgccgcaaaaaagggaataagggcgacacggaaatgttgaatactcatactcttcctttttcaatattattgaagcatttatcagggttattgtctcatgagcggatacatatttgaatgtatttagaaaaataaacaaataggggttccgcgcacatttccccgaaaagtgccacctgacgtctaagaaaccattattatcatgacattaacctataaaaataggcgtatcacgaggcccttaggccaaataggccgttcagatccttccgtatttagccagtatgttctctagtgtggttcgttgtttttgcgtgagccatgagaacgaaccattgagatcatgcttactttgcatgtcactcaaaaattttgcctcaaaactggtgagctgaatttttgcagttaaagcatcgtgtagtgtttttcttagtccgttacgtaggtaggaatctgatgtaatggttgttggtattttgtcaccattcatttttatctggttgttctcaagttcggttacgagatccatttgtctatctagttcaacttggaaaatcaacgtatcagtcgggcggcctcgcttatcaaccaccaatttcatattgctgtaagtgtttaaatctttacttattggtttcaaaacccattggttaagccttttaaactcatggtagttattttcaagcattaacatgaacttaaattcatcaaggctaatctctatatttgccttgtgagttttcttttgtgttagttcttttaataaccactcataaatcctcatagagtatttgttttcaaaagacttaacatgttccagattatattttatgaatttttttaactggaaaagataaggcaatatctcttcactaaaaactaattctaatttttcgcttgagaacttggcatagtttgtccactggaaaatctcaaagcctttaaccaaaggattcctgatttccacagttctcgtcatcagctctctggttgctttagctaatacaccataagcattttccctactgatgttcatcatctgagcgtattggttataagtgaacgataccgtccgttctttccttgtagggttttcaatcgtggggttgagtagtgccacacagcataaaattagcttggtttcatgctccgttaagtcatagcgactaatcgctagttcatttgctttgaaaacaactaattcagacatacatctcaattggtctaggtgattttaatcactataccaattgagatgggctagtcaatgataattactagtccttttcctttgagttgtgggtatctgtaaattctgctagacctttgctggaaaacttgtaaattctgctagaccctctgtaaattccgctagacctttgtgtgttttttttgtttatattcaagtggttataatttatagaataaagaaagaataaaaaaagataaaaagaatagatcccagccctgtgtataactcactactttagtcagttccgcagtattacaaaaggatgtcgcaaacgctgtttgctcctctacaaaacagaccttaaaaccctaaaggcttaagtagcaccctcgcaagctcgggcaaatcgctgaatattccttttgtctccgaccatcaggcacctgagtcgctgtctttttcgtgacattcagttcgctgcgctcacggctctggcagtgaatgggggtaaatggcactacaggcgccttttatggattcatgcaaggaaactacccataatacaagaaaagcccgtcacgggcttctcagggcgttttatggcgggtctgctatgtggtgctatctgactttttgctgttcagcagttcctgccctctgattttccagtctgaccacttcggattatcccgtgacaggtcattcagactggctaatgcacccagtaaggcagcggtatcatcaacaggcttacccgtcttactgtcaagaggacatccggtcagataaccgtcatcttcggctactgtctagggcggcggatttgtcctactcaggagagcgttcaccgacaaacaacagataaaacgaaaggcccagtctttcgactgagcctttcgttttatttgatgcactagtgccgatcatattcaataacccttaatataacttcgtataatgtatgctatacgaagttattaggtctgaagaggagtttacgtcccatatggagtcccgctcagaagaactcgtcaagaaggcgatagaaggcgatgcgctgcgaatcgggagcggcgataccgtaaagcacgaggaagcggtcagcccattcgccgccaagctcttcagcaatatcacgggtagccaacgctatgtcctgatagcggtccgccacacccagccggccacagtcgatgaatccagaaaagcggccattttccaccatgatattcggcaagcaggcatcgccatgggtcacgacgagatcctcgccgtcgggcatgcgcgccttgagcctggcgaacagttcggccggcgcgagcccctgatgctcttcgtccagatcatcctgatcgacaagaccggcttccatccgagtacgtgctcgctcgatgcgatgtttcgcttggtggtcgaatgggcaggtagccggatcaagcgtatgcagccgccgcattgcatcagccatgatggatactttctcggcaggagcaaggtgagatgacaggagatcctgccccggcacttcgcccaatagcagccagtcccttcccgcttcagtgacaacgtcgagcacagctgcgcaaggaacgcccgtcgtggccagccacgatagccgcgctgcctcgtcctgcagttcattcagggcaccggacaggtcggtcttgacaaaaagaaccgggcgcccctgcgctgacagccggaacacggcggcatcagagcagccgattgtctgttgtgcccagtcatagccgaatagcctctccacccaagcggccggagaacctgcgtgcaatccatcttgttcaatcatgcgaaacgatcctcatcctgtctcttgatcagatcctgatcccctgcgccatcagatccttggcggcaagaaagccatccagtttactttgcagggcttcccaaccttaccagagggcgccccagctggcaattccgacgtcattgcgttgctagccaagcttaggatccggaacccttaatataacttcgtataatgtatgctatacgaagttattaggtccctcgaagaggttcactagctatctagagcttggactcctgttgatagatccagtaatgacctcagaactccatctggatttgttcagaacgctcggttgccgccgggcgttttttattggtgagaatccaagcccgggaaacgggatcctgatcttgatcaggctgtgggtcaggccactcttggcatcgacaccaatgtgggccttcatgccaaagtgccactgattgcctttcttggtctgatgcatctccggatcgcgttgctgctctttgttcttggtcgagctgggtgcctcaatgatggtggcatcgaccaaggtgccttgagtcatcatgacgcctgcttcggccagccagcgattgatggtcttgaacaattggcgggccagttgatgctgctccagcaggtggcggaaattcatgatggtggtgcggtccggcaaggcgctatccagggataaccgggcaaacagacgcatggaggcgatttcgtacagagcatcttccatcgcgccatcgctcaggttgtaccaatgctgcatgcagtgaatgcgtagcatggtttccagcggataaggtcgccggccattaccagccttggggtaaaacggctcgatgacttccaccatgttttgccatggcagaatctgctccatgcgggacaagaaaatctcttttctggtctgacggcgcttactgctgaattcactgtcggcgaaggtaagttgatgactcatgatgaaccctgttctatggctccagatgacaaacatgatctcatatcagggacttgttcgcaccttccttagcacgttaattatctatcgtgtatatggaggggatctagaatgaaaaaaataatgctagtttttattacacttatattagttagtctaccaattgcgcaacaaactgaagcaaaggatgcatctgcattcaataaagaaaattcaatttcatccatggcaccaccagcatctccgcctgcaagtcctaagacgccaatcgaaaagaaacacgcggatgaaatcgataagtatatacaaggattggactacaataaaaacaatgtattagtataccacggagatgcagtgacaaatgtgccgccaagaaaaggttacaaagatggaaatgaatatattgttgtggagaaaaagaagaaatccatcaatcaaaataatgcagacattcaagttgtgaatgcaatttcgagcctaacctatccaggtgctctcgtaaaagcgaattcggaattagtagaaaatcaaccagatgttctccctgtaaaacgtgattcattaacactcagcattgatttgccaggtatgactaatcaagacaataaaatcgttgtaaaaaatgccactaaatcaaacgttaacaacgcagtaaatacattagtggaaagatggaatgaaaaatatgctcaagcttatccaaatgtaagtgcaaaaattgattatgatgacgaaatggcttacagtgaatcacaattaattgcgaaatttggtacagcatttaaagctgtaaataatagcttgaatgtaaacttcggcgcaatcagtgaagggaaaatgcaagaagaagtcattagttttaaacaaatttactataacgtgaatgttaatgaacctacaagaccttccagatttttcggcaaagctgttactaaagagcagttgcaagcgcttggagtgaatgcagaaaatcctcctgcatatatctcaagtgtggcgtatggccgtcaagtttatttgaaattatcaactaattcccatagtactaaagtaaaagctgcttttgatgctgccgtaagcggaaaatctgtctcaggtgatgtagaactaacaaatatcatcaaaaattcttccttcaaagccgtaatttacggaggttccgcaaaagatgaagttcaaatcatcgacggcaacctcggagacttacgagatattttgaaaaaaggcgctacttttaatcgagaaacaccaggagttcccattgcttatacaacaaacttcctaaaagacaatgaattagctgttattaaaaacaactcagaatatattgaaacaacttcaaaagcttatacagatggaaaaattaacatcgatcactctggaggatacgttgctcaattcaacatttcttgggatgaagtaaattatgatcctgaaggtaacgaaattgttcaacataaaaactggagcgaaaacaataaaagtaagctagctcatttcacatcgtccatctatttgccaggtaacgcgagaaatattaatgtttacgctaaagaatgcactggtttagcttgggaatggtggagaacggtaattgatgaccggaacttaccacttgtgaaaaatagaaatatctccatctggggcaccacgctttatccgaaatatagtaataaagtagataatccaatcgaataagtcgacctcgaggactagtgaacctcttcgagggacctaataacttcgtatagcatacattatacgaagttatattaagggttattgaatatgatcggctcgagattacttcgcattgcaatcagctacggactcaagcttacgtcaggtcatacgatgaaggcgataagtcgcgtaagttgctagcccacgcggctcaccttcacgggtgggcctttcttcgcgatccacatg

SEQ ID NO: 56 - DNA, 5456 bp, synthetic construct
  source 1..5456: mol_type = other DNA
catggtcatagctgtttcctttaatgcccatggcgtttaccaatgcttaatcagtgaggcacctatctcagcgatctgtctatttcgttcatccatagttgcctgactccccgtcgtgtagataactacgatacgggagggcttaccatctggccccagtgctgcaatgataccgcgacttccacgctcaccggctccagatttatcagcaataaaccagccagccggaagggccgagcgcagaagtggtcctgcaactttatccgcctccatccagtctattaattgttgccgggaagctagagtaagtagttcgccagttaatagtttgcgcaacgttgttgccattgctacaggcatcgtggtgtcacgctcgtcgtttggtatggcttcattcagctccggttcccaacgatcaaggcgagttacatgatcccccatgttgtgcaaaaaagcggttagctccttcggtcctccgatcgttgtcagaagtaagttggccgcagtgttatcactcatggttatggcagcactgcataattctcttactgtcatgccatccgtaagatgcttttctgtgactggtgagtactcaaccaagtcattctgagaatagtgtatgcggcgaccgagttgctcttgcccggcgtcaatacgggataataccgcgccacatagcagaactttaaaagtgctcatcattggaaaacgttcttcggggcgaaaactctcaaggatcttaccgctgttgagatccagttcgatgtaacccactcgtgcacccaactgatcttcagcatcttttactttcaccagcgtttctgggtgagcaaaaacaggaaggcaaaatgccgcaaaaaagggaataagggcgacacggaaatgttgaatactcatactcttcctttttcaatattattgaagcatttatcagggttattgtctcatgagcggatacatatttgaatgtatttagaaaaataaacaaataggggttccgcgcacatttccccgaaaagtgccacctgacgtctaagaaaccattattatcatgacattaacctataaaaataggcgtatcacgaggcccttaggccaaataggccgttcagatccttccgtatttagccagtatgttctctagtgtggttcgttgtttttgcgtgagccatgagaacgaaccattgagatcatgcttactttgcatgtcactcaaaaattttgcctcaaaactggtgagctgaatttttgcagttaaagcatcgtgtagtgtttttcttagtccgttacgtaggtaggaatctgatgtaatggttgttggtattttgtcaccattcatttttatctggttgttctcaagttcggttacgagatccatttgtctatctagttcaacttggaaaatcaacgtatcagtcgggcggcctcgcttatcaaccaccaatttcatattgctgtaagtgtttaaatctttacttattggtttcaaaacccattggttaagccttttaaactcatggtagttattttcaagcattaacatgaacttaaattcatcaaggctaatctctatatttgccttgtgagttttcttttgtgttagttcttttaataaccactcataaatcctcatagagtatttgttttcaaaagacttaacatgttccagattatattttatgaatttttttaactggaaaagataaggcaatatctcttcactaaaaactaattctaatttttcgcttgagaacttggcatagtttgtccactggaaaatctcaaagcctttaaccaaaggattcctgatttccacagttctcgtcatcagctctctggttgctttagctaatacaccataagcattttccctactgatgttcatcatctgagcgtattggttataagtgaacgataccgtccgttctttccttgtagggttttcaatcgtggggttgagtagtgccacacagcataaaattagcttggtttcatgctccgttaagtcatagcgactaatcgctagttcatttgctttgaaaacaactaattcagacatacatctcaattggtctaggtgattttaatcactataccaattgagatgggctagtcaatgataattactagtccttttcctttgagttgtgggtatctgtaaattctgctagacctttgctggaaaacttgtaaattctgctagaccctctgtaaattccgctagacctttgtgtgttttttttgtttatattcaagtggttataatttatagaataaagaaagaataaaaaaagataaaaagaatagatcccagccctgtgtataactcactactttagtcagttccgcagtattacaaaaggatgtcgcaaacgctgtttgctcctctacaaaacagaccttaaaaccctaaaggcttaagtagcaccctcgcaagctcgggcaaatcgctgaatattccttttgtctccgaccatcaggcacctgagtcgctgtctttttcgtgacattcagttcgctgcgctcacggctctggcagtgaatgggggtaaatggcactacaggcgccttttatggattcatgcaaggaaactacccataatacaagaaaagcccgtcacgggcttctcagggcgttttatggcgggtctgctatgtggtgctatctgactttttgctgttcagcagttcctgccctctgattttccagtctgaccacttcggattatcccgtgacaggtcattcagactggctaatgcacccagtaaggcagcggtatcatcaacaggcttacccgtcttactgtcaagaggacatccggtcagataaccgtcatcttcggctactgtctagggcggcggatttgtcctactcaggagagcgttcaccgacaaacaacagataaaacgaaaggcccagtctttcgactgagcctttcgttttatttgatgcactagtgccgatcatattcaataacccttaatataacttcgtataatgtatgctatacgaagttattaggtctgaagaggagtttacgtcccatatggagtcccgcttacgccccgccctgccactcatcgcagtactgttgtaattcattaagcattctgccgacatggaagccatcacagacggcatgatgaacctgaatcgccagcggcatcagcaccttgtcgccttgcgtataatatttgcccatggtgaaaacgggggcgaagaagttgtccatattggccacgtttaaatcaaaactggtgaaactcacccagggattggctgagacgaaaaacatattctcaataaaccctttagggaaataggccaggttttcaccgtaacacgccacatcttgcgaatatatgtgtagaaactgccggaaatcgtcgtggtattcactccagagcgatgaaaacgtttcagtttgctcatggaaaacggtgtaacaagggtgaacactatcccatatcaccagctcaccgtctttcattgccatacgaaattccggatgagcattcatcaggcgggcaagaatgtgaataaaggccggataaaacttgtgcttatttttctttacggtctttaaaaaggccgtaatatccagctgaacggtctggttataggtacattgagcaactgactgaaatgcctcaaaatgttctttacgatgccattgggatatatcaacggtggtatatccagtgatttttttctccattttagcttccttagctcctgaaaatctcgataactcaaaaaatacgcccggtagtgatcttatttcattatggtgaaagttggaacctcttacgtgccgatcagacgtcattgcgttgctagccaagcttaggatccggaacccttaatataacttcgtataatgtatgctatacgaagttattaggtccctcgaagaggttcactagctatctagagcttggactcctgttgatagatccagtaatgacctcagaactccatctggatttgttcagaacgctcggttgccgccgggcgttttttattggtgagaatccaagcccgggaaacgggatcctgatcttgatcaaccgaggtcacaacatagtaaaagcgctattggtaatggtacaatcgcgcgtttacacttattcagaacgatttttttcaggagggcctacttgtcacacaggacggtaatgtcgtgcccggttattgagctgacacagcaacttattcgtcgcccctccctgagtccggatgacgcaggctgtcaggcattaatgattgaacgcctgcgtaaaatcggttttaccattgagcatatggattttggcgacacgcaaaatttttgggcatggcgtgggcgtggcgaaacgctggcgttcgccgggcatactgacgtcgtaccggctggcgatgtcgatcgctggatcaatccgccgtttgagcctacgattcgcgacggaatgttgttcggtcgcggcgcggcggatatgaaaggttcactggcggccatggtggtggctgctgaacgttttgttgcgcagcatcctcatcaccggggccgcctcgcatttttgattacctctgatgaggaagccagcgcaaaaaatggcaccgtaaaggtggttgaagcgctgatggcccgtaacgagcggctggattactgtctggtcggcgaaccttccagtactgaaattgtgggcgatgtcgtcaaaaacgggcgtcgcggttctctcacctgtaacctcactatccatggcgttcaggggcacgtcgcctatccgcatctggcggataaccctgttcatcgcgccgcgccttttcttaatgaactggtcgctatcgagtgggatcggggcaatgactttttcccggccaccagtatgcaggtagccaatatccaggcaggcaccggcagcaataatgtcattcccggcgaactgttcgtgcagtttaacttccgtttcagcacggaactgaccgatgagatgatcaaagagcgggtacatgcgctgcttgaaaagcatcagctacgctataccgtagactggtggctttccgggcagccgttcctgaccgcacgcggcaagctggtggacgcggtggtaaacgccattgagcactataatgaaattaaaccgcaattactgacgacgggcggtacgtccgacggacgttttatcgcccgtatgggagcgcaggtggtagaactggggccggtgaacgccaccattcataaaattaatgaatgtgtgaatgccgccgatctccagctactggcccgtatgtatcaacgcattatggaacagctcgtcgcccatcaccatcaccatcactaagattacttcgcattgcaatcagctacggactcaagcttacgtcaggtcatacgatgaaggcgataagtcgcgtaagttgctagcccacgcggctcaccttcacgggtgggcctttcttcgcgatccacatg

SEQ ID NO: 57 - DNA, 76 bp, synthetic construct
  source 1..76: mol_type = other DNA
ttcacagaaaagtgttgcccccttccatggcggaagggggacaaaggtgaatttgtcctactcaggagagcgttca

SEQ ID NO: 58 - DNA, 68 bp, synthetic construct
  source 1..68: mol_type = other DNA
tctgacgtacacagcaattttgcgttacctgttaatcgagattgaaacaccgaagaaaggcccacccg

SEQ ID NO: 59 - DNA, 72 bp, synthetic construct
  source 1..72: mol_type = other DNA
ttggtttcagtgaatcccgttatcagcagttttttgatgaggtgtagtctatttgtcctactcaggagagcg

SEQ ID NO: 60 - DNA, 68 bp, synthetic construct
  source 1..68: mol_type = other DNA
caatattttgccagccagtccatgcttatttcctcttaccggaacgctcacgaagaaaggcccacccg

SEQ ID NO: 61 - protein, 5 aa, synthetic construct
EEEEE

SEQ ID NO: 62 - DNA, 15 bp, synthetic construct
  source 1..15: mol_type = other DNA
gaagaagaagaagaa

SEQ ID NO: 63 - protein, 5 aa, synthetic construct
NNNNN

SEQ ID NO: 64 - DNA, 15 bp, synthetic construct
  source 1..15: mol_type = other DNA
aacaacaacaacaac

SEQ ID NO: 65 - protein, 5 aa, synthetic construct
QQQQQ

SEQ ID NO: 66 - DNA, 15 bp, synthetic construct
  source 1..15: mol_type = other DNA
cagcagcagcagcag

SEQ ID NO: 67 - protein, 5 aa, synthetic construct
KKKKK

SEQ ID NO: 68 - DNA, 15 bp, synthetic construct
  source 1..15: mol_type = other DNA
aagaagaagaagaag

SEQ ID NO: 69 - protein, 5 aa, synthetic construct
RRRRR

SEQ ID NO: 70 - DNA, 15 bp, synthetic construct
  source 1..15: mol_type = other DNA
cggcggcggcggcgg

SEQ ID NO: 71 - protein, 4 aa, synthetic construct
DDDD

SEQ ID NO: 72 - DNA, 12 bp, synthetic construct
  source 1..12: mol_type = other DNA
gatgatgatgat

SEQ ID NO: 73 - protein, 5 aa, synthetic construct
DDDDD

SEQ ID NO: 74 - DNA, 15 bp, synthetic construct
  source 1..15: mol_type = other DNA
gatgatgatgatgat

SEQ ID NO: 75 - protein, 6 aa, synthetic construct
DDDDDD

SEQ ID NO: 76 - DNA, 18 bp, synthetic construct
  source 1..18: mol_type = other DNA
gatgatgatgatgatgat

SEQ ID NO: 77 - protein, 7 aa, synthetic construct
DDDDDDD

SEQ ID NO: 78 - DNA, 21 bp, synthetic construct
  source 1..21: mol_type = other DNA
gatgatgatgatgatgatgat

SEQ ID NO: 79 - protein, 8 aa, synthetic construct
DDDDDDDD

SEQ ID NO: 80 - DNA, 24 bp, synthetic construct
  source 1..24: mol_type = other DNA
gatgatgatgatgatgatgatgat

SEQ ID NO: 81 - protein, 9 aa, synthetic construct
DDDDDDDDD

SEQ ID NO: 82 - DNA, 27 bp, synthetic construct
  source 1..27: mol_type = other DNA
gatgatgatgatgatgatgatgatgat

SEQ ID NO: 83 - protein, 10 aa, synthetic construct
DDDDDDDDDD

SEQ ID NO: 84 - DNA, 30 bp, synthetic construct
  source 1..30: mol_type = other DNA
gatgatgatgatgatgatgatgatgatgat

SEQ ID NO: 85 - protein, 5 aa, synthetic construct
DDDEE

SEQ ID NO: 86 - DNA, 15 bp, synthetic construct
  source 1..15: mol_type = other DNA
gatgatgatgaagaa

SEQ ID NO: 87 - protein, 6 aa, synthetic construct
DDDEEE

SEQ ID NO: 88 - DNA, 18 bp, synthetic construct
  source 1..18: mol_type = other DNA
gatgatgatgaagaagaa

SEQ ID NO: 89 - protein, 5 aa, synthetic construct
DEDED

SEQ ID NO: 90 - DNA, 15 bp, synthetic construct
  source 1..15: mol_type = other DNA
gatgaagatgaagat

SEQ ID NO: 91 - protein, 5 aa, synthetic construct
DDEDD

SEQ ID NO: 92 - DNA, 15 bp, synthetic construct
  source 1..15: mol_type = other DNA
gatgatgaagatgat

SEQ ID NO: 93 - protein, 6 aa, synthetic construct
DDEDDE

SEQ ID NO: 94 - DNA, 18 bp, synthetic construct
  source 1..18: mol_type = other DNA
gatgatgaagatgatgaa

SEQ ID NO: 95 - protein, 5 aa, synthetic construct
DDDNN

SEQ ID NO: 96 - DNA, 15 bp, synthetic construct
  source 1..15: mol_type = other DNA
gaagaagaaaacaac

SEQ ID NO: 97 - protein, 6 aa, synthetic construct
DDDNNN

SEQ ID NO: 98 - DNA, 18 bp, synthetic construct
  source 1..18: mol_type = other DNA
gaagaagaaaacaacaac